European Patent Application EP 4 621 056 A1, published September 24, 2025. Title: BLOOD COAGULATION FACTOR VIII VARIANT PRODUCING CELLS FOR EX VIVO GENE THERAPY. Applicant: セルジェンテック株式会社. The sequence listing filed with the application follows.

SEQUENCE LISTING (35 sequences)

SEQ ID NO: 1 - protein, 2351 aa, Homo sapiens
MQIELSTCFFLCLLRFCFSATRRYYLGAVELSWDYMQSDLGELPVDARFPPRVPKSFPFNTSVVYKKTLFVEFTDHLFNIAKPRPPWMGLLGPTIQAEVYDTVVITLKNMASHPVSLHAVGVSYWKASEGAEYDDQTSQREKEDDKVFPGGSHTYVWQVLKENGPMASDPLCLTYSYLSHVDLVKDLNSGLIGALLVCREGSLAKEKTQTLHKFILLFAVFDEGKSWHSETKNSLMQDRDAASARAWPKMHTVNGYVNRSLPGLIGCHRKSVYWHVIGMGTTPEVHSIFLEGHTFLVRNHRQASLEISPITFLTAQTLLMDLGQFLLFCHISSHQHDGMEAYVKVDSCPEEPQLRMKNNEEAEDYDDDLTDSEMDVVRFDDDNSPSFIQIRSVAKKHPKTWVHYIAAEEEDWDYAPLVLAPDDRSYKSQYLNNGPQRIGRKYKKVRFMAYTDETFKTREAIQHESGILGPLLYGEVGDTLLIIFKNQASRPYNIYPHGITDVRPLYSRRLPKGVKHLKDFPILPGEIFKYKWTVTVEDGPTKSDPRCLTRYYSSFVNMERDLASGLIGPLLICYKESVDQRGNQIMSDKRNVILFSVFDENRSWYLTENIQRFLPNPAGVQLEDPEFQASNIMHSINGYVFDSLQLSVCLHEVAYWYILSIGAQTDFLSVFFSGYTFKHKMVYEDTLTLFPFSGETVFMSMENPGLWILGCHNSDFRNRGMTALLKVSSCDKNTGDYYEDSYEDISAYLLSKNNAIEPRSFSQNSRHPSTRQKQFNATTIPENDIEKTDPWFAHRTPMPKIQNVSSSDLLMLLRQSPTPHGLSLSDLQEAKYETFSDDPSPGAIDSNNSLSEMTHFRPQLHHSGDMVFTPESGLQLRLNEKLGTTAATELKKLDFKVSSTSNNLISTIPSDNLAAGTDNTSSLGPPSMPVHYDSQLDTTLFGKKSSPLTESGGPLSLSEENNDSKLLESGLMNSQESSWGKNVSSTESGRLFKGKRAHGPALLTKDNALFKVSISLLKTNKTSNNSATNRKTHIDGPSLLIENSPSVWQNILESDTEFKKVTPLIHDRMLMDKNATALRLNHMSNKTTSSKNMEMVQQKKEGPIPPDAQNPDMSFFKMLFLPESARWIQRTHGKNSLNSGQGPSPKQLVSLGPEKSVEGQNFLSEKNKVVVGKGEFTKDVGLKEMVFPSSRNLFLTNLDNLHENNTHNQEKKIQEEIEKKETLIQENVVLPQIHTVTGTKNFMKNLFLLSTRQNVEGSYDGAYAPVLQDFRSLNDSTNRTKKHTAHFSKKGEEENLEGLGNQTKQIVEKYACTTRISPNTSQQNFVTQRSKRALKQFRLPLEETELEKRIIVDDTSTQWSKNMKHLTPSTLTQIDYNEKEKGAITQSPLSDCLTRSHSIPQANRSPLPIAKVSSFPSIRPIYLTRVLFQDNSSHLPAASYRKKDSGVQESSHFLQGAKKNNLSLAILTLEMTGDQREVGSLGTSATNSVTYKKVENTVLPKPDLPKTSGKVELLPKVHIYQKDLFPTETSNGSPGHLDLVEGSLLQGTEGAIKWNEANRPGKVPFLRVATESSAKTPSKLLDPLAWDNHYGTQIPKEEWKSQEKSPEKTAFKKKDTILSLNACESNHAIAAINEGQNKPEIEVTWAKQGRTERLCSQNPPVLKRHQREITRTTLQSDQEEIDYDDTISVEMKKEDFDIYDEDENQSPRSFQKKTRHYFIAAVERLWDYGMSSSPHVLRNRAQSGSVPQFKKVVFQEFTDGSFTQPLYRGELNEHLGLLGPYIRAEVEDNIMVTFRNQASRPYSFYSSLISYEEDQRQGAEPRKNFVKPNETKTYFWKVQHHMAPTKDEFDCKAWAYFSDVDLEKDVHSGLIGPLLVCHTNTLNPAHGRQVTVQEFALFFTIFDETKSWYFTENMERNCRAPCNIQMEDPTFKENYRFHAINGYIMDTLPGLVMAQDQRIRWYLLSMGSNENIHSIHFSGHVFTVRKKEEYKMALYNLYPGVFETVEMLPSKAGIWRVECLIGEHLHAGMSTLFLVYSNKCQTPLGMASGHIRDFQITASGQYGQWAPKLARLHYSGSINAWSTKEPFSWIKVDLLAPMIIHGIKTQGARQKFSSLYISQFIIMYSLDGKKWQTYRGNSTGTLMVFFGNVDSSGIKHNIFNPPIIARYIRLHPTHYSIRSTLRMELMGCDLNSCSMPLGMESKAISDAQITASSYFTNMFATWSPSKARLHLQGRSNAWRPQVNNPKEWLQVDFQKTMKVTGVTTQGVKSLLTSMYVKEFLISSSQDGHQWTLFFQNGKVKVFQGNQDSFTPVVNSLDPPLLTRYLRIHPQSWVHQIALRMEVLGCEAQDLY

SEQ ID NO: 2 - protein, 1607 aa, synthetic construct
MQIELSTCFFLCLLRFCFSATRRYYLGAVELSWDYMQSDLGELPVDARFPPRVPKSFPFNTSVVYKKTLFVEFTDHLFNIAKPRPPWMGLLGPTIQAEVYDTVVITLKNMASHPVSLHAVGVSYWKASEGAEYDDQTSQREKEDDKVFPGGSHTYVWQVLKENGPMASDPLCLTYSYLSHVDLVKDLNSGLIGALLVCREGSLAKEKTQTLHKFILLFAVFDEGKSWHSETKNSLMQDRDAASARAWPKMHTVNGYVNRSLPGLIGCHRKSVYWHVIGMGTTPEVHSIFLEGHTFLVRNHRQASLEISPITFLTAQTLLMDLGQFLLFCHISSHQHDGMEAYVKVDSCPEEPQLRMKNNEEAEDYDDDLTDSEMDVVRFDDDNSPSFIQIRSVAKKHPKTWVHYIAAEEEDWDYAPLVLAPDDRSYKSQYLNNGPQRIGRKYKKVRFMAYTDETFKTREAIQHESGILGPLLYGEVGDTLLIIFKNQASRPYNIYPHGITDVRPLYSRRLPKGVKHLKDFPILPGEIFKYKWTVTVEDGPTKSDPRCLTRYYSSFVNMERDLASGLIGPLLICYKESVDQRGNQIMSDKRNVILFSVFDENRSWYLTENIQRFLPNPAGVQLEDPEFQASNIMHSINGYVFDSLQLSVCLHEVAYWYILSIGAQTDFLSVFFSGYTFKHKMVYEDTLTLFPFSGETVFMSMENPGLWILGCHNSDFRNRGMTALLKVSSCDKNTGDYYEDSYEDISAYLLSKNNAIEPRSFSQNSRHPSTRQKQFNATTIPENDIEKTDPWFAHRTPMPKIQNVSSSDLLMLLRQSPTPHGLSLSDLQEAKYETFSDDPSPGAIDSNNSLSEMTHFRPQLHHSGDMVFTPESGLQLRLNEKLGTTAATELKKLDFKVSSTSNNLISTIPSDNLAAGTDNTSSREITRTTLQSDQEEIDYDDTISVEMKKEDFDIYDEDENQSPRSFQKKTRHYFIAAVERLWDYGMSSSPHVLRNRAQSGSVPQFKKVVFQEFTDGSFTQPLYRGELNEHLGLLGPYIRAEVEDNIMVTFRNQASRPYSFYSSLISYEEDQRQGAEPRKNFVKPNETKTYFWKVQHHMAPTKDEFDCKAWAYFSDVDLEKDVHSGLIGPLLVCHTNTLNPAHGRQVTVQEFALFFTIFDETKSWYFTENMERNCRAPCNIQMEDPTFKENYRFHAINGYIMDTLPGLVMAQDQRIRWYLLSMGSNENIHSIHFSGHVFTVRKKEEYKMALYNLYPGVFETVEMLPSKAGIWRVECLIGEHLHAGMSTLFLVYSNKCQTPLGMASGHIRDFQITASGQYGQWAPKLARLHYSGSINAWSTKEPFSWIKVDLLAPMIIHGIKTQGARQKFSSLYISQFIIMYSLDGKKWQTYRGNSTGTLMVFFGNVDSSGIKHNIFNPPIIARYIRLHPTHYSIRSTLRMELMGCDLNSCSMPLGMESKAISDAQITASSYFTNMFATWSPSKARLHLQGRSNAWRPQVNNPKEWLQVDFQKTMKVTGVTTQGVKSLLTSMYVKEFLISSSQDGHQWTLFFQNGKVKVFQGNQDSFTPVVNSLDPPLLTRYLRIHPQSWVHQIALRMEVLGCEAQDLY

SEQ ID NO: 3 - protein, 1652 aa, synthetic construct
MQIELSTCFFLCLLRFCFSATRRYYLGAVELSWDYMQSDLGELPVDARFPPRVPKSFPFNTSVVYKKTLFVEFTDHLFNIAKPRPPWMGLLGPTIQAEVYDTVVITLKNMASHPVSLHAVGVSYWKASEGAEYDDQTSQREKEDDKVFPGGSHTYVWQVLKENGPMASDPLCLTYSYLSHVDLVKDLNSGLIGALLVCREGSLAKEKTQTLHKFILLFAVFDEGKSWHSETKNSLMQDRDAASARAWPKMHTVNGYVNRSLPGLIGCHRKSVYWHVIGMGTTPEVHSIFLEGHTFLVRNHRQASLEISPITFLTAQTLLMDLGQFLLFCHISSHQHDGMEAYVKVDSCPEEPQLRMKNNEEAEDYDDDLTDSEMDVVRFDDDNSPSFIQIRSVAKKHPKTWVHYIAAEEEDWDYAPLVLAPDDRSYKSQYLNNGPQRIGRKYKKVRFMAYTDETFKTREAIQHESGILGPLLYGEVGDTLLIIFKNQASRPYNIYPHGITDVRPLYSRRLPKGVKHLKDFPILPGEIFKYKWTVTVEDGPTKSDPRCLTRYYSSFVNMERDLASGLIGPLLICYKESVDQRGNQIMSDKRNVILFSVFDENRSWYLTENIQRFLPNPAGVQLEDPEFQASNIMHSINGYVFDSLQLSVCLHEVAYWYILSIGAQTDFLSVFFSGYTFKHKMVYEDTLTLFPFSGETVFMSMENPGLWILGCHNSDFRNRGMTALLKVSSCDKNTGDYYEDSYEDISAYLLSKNNAIEPRSFSQNSRHPSTRQKQFNATTIPENDIEKTDPWFAHRTPMPKIQNVSSSDLLMLLRQSPTPHGLSLSDLQEAKYETFSDDPSPGAIDSNNSLSEMTHFRPQLHHSGDMVFTPESGLQLRLNEKLGTTAATELKKLDFKVSSTSNNLISTIPSDNLAAGTDNTSSLGPPSMPVHYDSQLDTTLFGKKSSPLTESGGPLSLSEENNDSKLTREITRTTLQSDQEEIDYDDTISVEMKKEDFDIYDEDENQSPRSFQKKTRHYFIAAVERLWDYGMSSSPHVLRNRAQSGSVPQFKKVVFQEFTDGSFTQPLYRGELNEHLGLLGPYIRAEVEDNIMVTFRNQASRPYSFYSSLISYEEDQRQGAEPRKNFVKPNETKTYFWKVQHHMAPTKDEFDCKAWAYFSDVDLEKDVHSGLIGPLLVCHTNTLNPAHGRQVTVQEFALFFTIFDETKSWYFTENMERNCRAPCNIQMEDPTFKENYRFHAINGYIMDTLPGLVMAQDQRIRWYLLSMGSNENIHSIHFSGHVFTVRKKEEYKMALYNLYPGVFETVEMLPSKAGIWRVECLIGEHLHAGMSTLFLVYSNKCQTPLGMASGHIRDFQITASGQYGQWAPKLARLHYSGSINAWSTKEPFSWIKVDLLAPMIIHGIKTQGARQKFSSLYISQFIIMYSLDGKKWQTYRGNSTGTLMVFFGNVDSSGIKHNIFNPPIIARYIRLHPTHYSIRSTLRMELMGCDLNSCSMPLGMESKAISDAQITASSYFTNMFATWSPSKARLHLQGRSNAWRPQVNNPKEWLQVDFQKTMKVTGVTTQGVKSLLTSMYVKEFLISSSQDGHQWTLFFQNGKVKVFQGNQDSFTPVVNSLDPPLLTRYLRIHPQSWVHQIALRMEVLGCEAQDLY

SEQ ID NO: 4 - protein, 1670 aa, synthetic construct
MQIELSTCFFLCLLRFCFSATRRYYLGAVELSWDYMQSDLGELPVDARFPPRVPKSFPFNTSVVYKKTLFVEFTDHLFNIAKPRPPWMGLLGPTIQAEVYDTVVITLKNMASHPVSLHAVGVSYWKASEGAEYDDQTSQREKEDDKVFPGGSHTYVWQVLKENGPMASDPLCLTYSYLSHVDLVKDLNSGLIGALLVCREGSLAKEKTQTLHKFILLFAVFDEGKSWHSETKNSLMQDRDAASARAWPKMHTVNGYVNRSLPGLIGCHRKSVYWHVIGMGTTPEVHSIFLEGHTFLVRNHRQASLEISPITFLTAQTLLMDLGQFLLFCHISSHQHDGMEAYVKVDSCPEEPQLRMKNNEEAEDYDDDLTDSEMDVVRFDDDNSPSFIQIRSVAKKHPKTWVHYIAAEEEDWDYAPLVLAPDDRSYKSQYLNNGPQRIGRKYKKVRFMAYTDETFKTREAIQHESGILGPLLYGEVGDTLLIIFKNQASRPYNIYPHGITDVRPLYSRRLPKGVKHLKDFPILPGEIFKYKWTVTVEDGPTKSDPRCLTRYYSSFVNMERDLASGLIGPLLICYKESVDQRGNQIMSDKRNVILFSVFDENRSWYLTENIQRFLPNPAGVQLEDPEFQASNIMHSINGYVFDSLQLSVCLHEVAYWYILSIGAQTDFLSVFFSGYTFKHKMVYEDTLTLFPFSGETVFMSMENPGLWILGCHNSDFRNRGMTALLKVSSCDKNTGDYYEDSYEDISAYLLSKNNAIEPRSFSQNSRHPSTRQKQFNATTIPENDIEKTDPWFAHRTPMPKIQNVSSSDLLMLLRQSPTPHGLSLSDLQEAKYETFSDDPSPGAIDSNNSLSEMTHFRPQLHHSGDMVFTPESGLQLRLNEKLGTTAATELKKLDFKVSSTSNNLISTIPSDNLAAGTDNTSSLGPPSMPVHYDSQLDTTLFGKKSSPLTESGGPLSLSEENNDSKLLESGLMNSQESSWGKNVSSREITRTTLQSDQEEIDYDDTISVEMKKEDFDIYDEDENQSPRSFQKKTRHYFIAAVERLWDYGMSSSPHVLRNRAQSGSVPQFKKVVFQEFTDGSFTQPLYRGELNEHLGLLGPYIRAEVEDNIMVTFRNQASRPYSFYSSLISYEEDQRQGAEPRKNFVKPNETKTYFWKVQHHMAPTKDEFDCKAWAYFSDVDLEKDVHSGLIGPLLVCHTNTLNPAHGRQVTVQEFALFFTIFDETKSWYFTENMERNCRAPCNIQMEDPTFKENYRFHAINGYIMDTLPGLVMAQDQRIRWYLLSMGSNENIHSIHFSGHVFTVRKKEEYKMALYNLYPGVFETVEMLPSKAGIWRVECLIGEHLHAGMSTLFLVYSNKCQTPLGMASGHIRDFQITASGQYGQWAPKLARLHYSGSINAWSTKEPFSWIKVDLLAPMIIHGIKTQGARQKFSSLYISQFIIMYSLDGKKWQTYRGNSTGTLMVFFGNVDSSGIKHNIFNPPIIARYIRLHPTHYSIRSTLRMELMGCDLNSCSMPLGMESKAISDAQITASSYFTNMFATWSPSKARLHLQGRSNAWRPQVNNPKEWLQVDFQKTMKVTGVTTQGVKSLLTSMYVKEFLISSSQDGHQWTLFFQNGKVKVFQGNQDSFTPVVNSLDPPLLTRYLRIHPQSWVHQIALRMEVLGCEAQDLY

SEQ ID NO: 5 - protein, 1652 aa, synthetic construct
MQIELSTCFFLCLLRFCFSATRRYYLGAVELSWDYMQSDLGELPVDARFPPRVPKSFPFNTSVVYKKTLFVEFTDHLFNIAKPRPPWMGLLGPTIQAEVYDTVVITLKNMASHPVSLHAVGVSYWKASEGAEYDDQTSQREKEDDKVFPGGSHTYVWQVLKENGPMASDPLCLTYSYLSHVDLVKDLNSGLIGALLVCREGSLAKEKTQTLHKFILLFAVFDEGKSWHSETKNSLMQDRDAASARAWPKMHTVNGYVNRSLPGLIGCHRKSVYWHVIGMGTTPEVHSIFLEGHTFLVRNHRQASLEISPITFLTAQTLLMDLGQFLLFCHISSHQHDGMEAYVKVDSCPEEPQLRMKNNEEAEDYDDDLTDSEMDVVRFDDDNSPSFIQIRSVAKKHPKTWVHYIAAEEEDWDYAPLVLAPDDRSYKSQYLNNGPQRIGRKYKKVRFMAYTDETFKTREAIQHESGILGPLLYGEVGDTLLIIFKNQASRPYNIYPHGITDVRPLYSRRLPKGVKHLKDFPILPGEIFKYKWTVTVEDGPTKSDPRCLTRYYSSFVNMERDLASGLIGPLLICYKESVDQRGNQIMSDKRNVILFSVFDENRSWYLTENIQRFLPNPAGVQLEDPEFQASNIMHSINGYVFDSLQLSVCLHEVAYWYILSIGAQTDFLSVFFSGYTFKHKMVYEDTLTLFPFSGETVFMSMENPGLWILGCHNSDFRNRGMTALLKVSSCDKNTGDYYEDSYEDISAYLLSKNNAIETRSFSQNSRHPSTRQKQFNATTIPENDIEKTDPWFAHRTPMPKIQNVSSSDLLMLLRQSPTPHGLSLSDLQEAKYETFSDDPSPGAIDSNNSLSEMTHFRPQLHHSGDMVFTPESGLQLRLNEKLGTTAATELKKLDFKVSSTSNNLISTIPSDNLAAGTDNTSSLGPPSMPVHYDSQLDTTLFGKKSSPLTESGGPLSLSEENNDSKLTREITRTTLQSDQEEIDYDDTISVEMKKEDFDIYDEDENQSPRSFQKKTRHYFIAAVERLWDYGMSSSPHVLRNRAQSGSVPQFKKVVFQEFTDGSFTQPLYRGELNEHLGLLGPYIRAEVEDNIMVTFRNQASRPYSFYSSLISYEEDQRQGAEPRKNFVKPNETKTYFWKVQHHMAPTKDEFDCKAWAYFSDVDLEKDVHSGLIGPLLVCHTNTLNPAHGRQVTVQEFALFFTIFDETKSWYFTENMERNCRAPCNIQMEDPTFKENYRFHAINGYIMDTLPGLVMAQDQRIRWYLLSMGSNENIHSIHFSGHVFTVRKKEEYKMALYNLYPGVFETVEMLPSKAGIWRVECLIGEHLHAGMSTLFLVYSNKCQTPLGMASGHIRDFQITASGQYGQWAPKLARLHYSGSINAWSTKEPFSWIKVDLLAPMIIHGIKTQGARQKFSSLYISQFIIMYSLDGKKWQTYRGNSTGTLMVFFGNVDSSGIKHNIFNPPIIARYIRLHPTHYSIRSTLRMELMGCDLNSCSMPLGMESKAISDAQITASSYFTNMFATWSPSKARLHLQGRSNAWRPQVNNPKEWLQVDFQKTMKVTGVTTQGVKSLLTSMYVKEFLISSSQDGHQWTLFFQNGKVKVFQGNQDSFTPVVNSLDPPLLTRYLRIHPQSWVHQIALRMEVLGCEAQDLY

SEQ ID NO: 6 - DNA, 4824 bp, synthetic construct
  source 1..4824: mol_type = other DNA
atgcagattgagctcagcacatgcttctttctctgtctgctgaggttctgcttcagcgccacaagaaggtactatctcggagctgtggaactgagctgggactatatgcaaagcgatctgggcgaactgcccgtggatgccagattcccccccagagtgcctaagtccttccctttcaacaccagcgtggtctataagaagacactgttcgtcgagttcacagaccatctgttcaacatcgctaagcctaggcctccttggatgggactgctgggccccaccatccaagccgaggtgtacgataccgtggtgatcacactcaaaaacatggcctcccaccccgtgtccctccatgctgtgggagtctcctactggaaggcttccgaaggagccgagtatgacgatcagaccagccaaagggagaaagaagacgacaaagtgttccccggcggatcccatacctacgtctggcaagtgctcaaagagaatggccccatggctagcgatcccctctgcctcacatattcctatctgagccatgtggatctcgtcaaggatctgaactccggactgattggagctctgctggtctgtagggaaggatctctggctaaagagaaaacccagaccctccacaagttcattctgctcttcgccgtgttcgacgagggaaaaagctggcacagcgagacaaagaacagcctcatgcaagacagagatgctgcttccgccagagcttggcccaagatgcacaccgtcaacggctacgtgaataggagcctccccggcctcattggctgccacagaaagtccgtgtactggcacgtgattggcatgggaaccacccccgaggtgcactccatcttcctcgagggacacacatttctcgtgaggaaccacagacaagccagcctcgagatcagccccattacctttctgaccgctcagacactgctcatggacctcggacaatttctgctgttctgccacatcagctcccaccagcacgatggcatggaggcttatgtcaaggtcgatagctgccccgaggaacctcagctgagaatgaagaacaatgaagaggccgaggactacgacgacgatctgaccgatagcgagatggatgtcgtgagattcgacgacgacaacagccctagctttatccagattaggagcgtggccaagaaacaccccaaaacatgggtgcactacattgccgctgaggaagaggactgggattatgctcctctggtgctcgcccccgacgataggagctacaagtcccaatatctgaacaacggccctcaaaggatcggaagaaaatacaaaaaggtgagattcatggcttacaccgacgagacctttaagacaagggaggccatccagcatgaatccggaattctgggacctctgctctacggagaggtgggagacacactgctcattatcttcaagaatcaagcctctaggccctacaacatctatcctcacggcattacagacgtcagacctctgtattccagaaggctccccaagggcgtcaaacatctcaaggactttcccattctgcccggcgaaatcttcaaatacaagtggacagtgaccgtcgaagatggccctaccaaatccgaccctaggtgtctgacaaggtactattcctcctttgtgaacatggagagggatctggccagcggcctcatcggccctctcctcatctgctataaagagagcgtcgatcagagaggcaatcagatcatgtccgacaaaaggaacgtcatcctcttctccgtcttcgacgagaatagaagctggtatctgaccgagaacatccagagattcctccctaaccccgccggcgtccagctggaggatcccgagtttcaagcctccaatatcatgcactccattaatggctacgtgttcgactctctgcagctctccgtctgtctgcatgaggtggcttattggtacattctgagcatcggcgctcagacagattttctgtccgtcttcttcagcggctatacattcaagcataagatggtctatgaggacaccctcacactgttccccttctccggcgagaccgtcttcatgagcatggaaaaccccggactctggattctcggctgccacaattccgatttcagaaataggggaatgaccgctctgctgaaggtgagcagctgtgacaagaacaccggcgattattatgaggacagctacgaggacatttccgcctatctgctctccaagaacaacgctatcgagcctaggagcttctcccaaaattctaggcacccttccacaaggcagaagcaatttaacgccaccaccatccccgagaacgacattgagaagacagacccttggttcgcccataggacacccatgcccaagattcagaacgtcagcagctccgatctgctcatgctgctcagacaatcccctacaccccatggactctctctgtccgatctccaagaggccaaatacgagaccttctccgatgacccctcccccggcgccattgattccaacaactccctctccgaaatgacccactttagaccccaactgcaccactccggcgacatggtctttacccccgaatccggactgcagctgaggctgaacgagaagctgggcaccacagccgccacagaactcaaaaaactggattttaaagtgtcctccaccagcaacaatctgatcagcaccatcccctccgacaacctcgccgctggaacagacaacacctccagcagggagatcacaagaacaacactgcagtccgaccaagaggaaattgactacgatgataccattagcgtggagatgaagaaggaagacttcgatatttacgacgaagatgagaatcagagccctaggtccttccagaagaaaaccagacactacttcatcgccgctgtcgaaaggctctgggactacggcatgtcctccagcccccatgtgctgaggaatagggctcagagcggctccgtgccccagttcaagaaggtcgtctttcaagagtttaccgacggaagctttacccagcctctgtataggggagagctcaacgagcatctgggactgctcggcccttatattagagccgaagtggaagataatatcatggtgacatttaggaaccaagcctctaggccttatagcttctacagctccctcatcagctatgaggaagaccaaagacaaggcgccgagcctaggaagaactttgtcaagcccaacgagaccaagacctacttttggaaggtgcagcatcacatggctcctaccaaggacgaatttgattgtaaggcttgggcctacttcagcgacgtcgatctggaaaaggacgtgcattccggactgatcggacccctcctcgtctgtcataccaatacactgaaccccgcccacggaaggcaagtgaccgtccaagagttcgctctgttcttcaccattttcgatgaaaccaagagctggtactttacagaaaacatggaaaggaattgtagggccccttgcaacattcaaatggaagatcctacctttaaggagaattataggtttcacgccatcaacggctatatcatggataccctccccggactggtcatggcccaagaccagaggattaggtggtatctgctgagcatgggatccaacgaaaacatccacagcatccatttctccggacacgtctttaccgtgaggaagaaggaggagtataagatggccctctataatctctatcccggcgtgttcgaaaccgtggaaatgctgccctccaaggccggcatttggagagtggagtgtctgattggcgaacatctgcatgccggaatgagcacactctttctcgtgtacagcaacaagtgtcaaacacctctgggcatggctagcggacacatcagagacttccaaattaccgcctccggacagtacggacaatgggcccctaaactcgctaggctccactactccggatccatcaatgcttggtccaccaaggagcctttcagctggatcaaggtggatctcctcgcccccatgatcatccatggcattaagacccaaggcgctagacagaaatttagcagcctctacatctcccagtttattatcatgtactctctggatggcaagaagtggcaaacctatagaggcaacagcaccggcacactgatggtgttcttcggaaacgtggacagctccggcattaagcataacatcttcaacccccccatcattgctaggtatattaggctgcaccccacccactatagcattaggtccacactgaggatggagctgatgggctgcgatctgaacagctgcagcatgcccctcggaatggagtccaaggccatcagcgatgctcagatcaccgctagctcctacttcacaaacatgttcgccacatggtccccttccaaagctaggctgcacctccaaggcagaagcaatgcttggaggccccaagtcaacaatcccaaggagtggctgcaagtggatttccagaagaccatgaaagtcaccggcgtcacaacccaaggcgtgaaatctctgctgacatccatgtacgtgaaggagtttctgatctccagctcccaagacggccatcaatggaccctctttttccagaacggcaaggtgaaagtgttccaaggcaaccaagacagctttacacccgtggtgaatagcctcgacccccctctcctcacaaggtacctcagaattcacccccaaagctgggtccaccagattgctctgagaatggaggtcctcggctgcgaagcccaagacctctattga

SEQ ID NO: 7 - DNA, 4959 bp, synthetic construct
  source 1..4959: mol_type = other DNA
atgcagatcgagctgtctacctgcttcttcctgtgcctgctgcggttctgcttcagcgccaccagaagatattacctgggcgccgtggaactgagctgggactacatgcagtctgacctgggagagctgcccgtggacgctagatttcctccaagagtgcccaagagcttccccttcaacacctccgtggtgtacaagaaaaccctgttcgtggaattcaccgaccacctgttcaatatcgccaagcctcggcctccttggatgggactgctgggacctacaattcaggccgaggtgtacgacaccgtggtcatcaccctgaagaacatggccagccatcctgtgtctctgcacgccgtgggagtgtcttactggaaggcttctgagggcgccgagtacgacgatcagacaagccagagagagaaagaggacgacaaggttttccctggcggcagccacacctatgtctggcaggtcctgaaagaaaacggccctatggcctccgatcctctgtgcctgacatacagctacctgagccacgtggacctggtcaaggacctgaattctggcctgatcggagccctgctcgtgtgtagagaaggcagcctggccaaagagaaaacccagacactgcacaagttcatcctgctgttcgccgtgttcgacgagggcaagagctggcacagcgagacaaagaacagcctgatgcaggacagggatgccgcctctgctagagcttggcctaagatgcacaccgtgaacggctacgtgaacagaagcctgcctggactgatcggctgccacagaaagtccgtgtactggcacgtgatcggcatgggcacaacacctgaggtgcacagcatctttctggaaggacacaccttcctcgtgcggaaccatagacaggccagcctggaaatcagccctatcaccttcctgaccgctcagaccctgctgatggatctgggccagtttctgctgttctgccacatcagctcccaccagcacgatggcatggaagcctacgtgaaggtggacagctgccccgaagaaccccagctgcggatgaagaacaacgaggaagccgaggactacgacgacgacctgaccgactctgagatggacgtcgtcagattcgacgacgataacagccccagcttcatccagatcagaagcgtggccaagaagcaccccaagacctgggtgcactatatcgccgccgaggaagaggactgggattacgctcctctggtgctggcccctgacgacagaagctacaagagccagtacctgaacaacggccctcagcggatcggccggaagtataagaaagtgcggttcatggcctacaccgacgagacattcaagaccagagaggccatccagcacgagagcggaattctgggccctctgctgtatggcgaagtgggcgatacactgctgatcatcttcaagaaccaggccagcagaccctacaacatctaccctcacggcatcaccgatgtgcggcccctgtattctagaaggctgcccaagggcgtgaagcacctgaaggacttccctatcctgcctggcgagatcttcaagtacaagtggaccgtgaccgtggaagatggccccaccaagagcgaccctagatgtctgacacggtactacagcagcttcgtgaacatggaacgcgacctggccagcggcctgattggacctctgctgatctgctacaaagaaagcgtggaccagcggggcaaccagatcatgagcgacaagcggaacgtgatcctgtttagcgtgttcgatgagaaccggtcctggtatctgaccgagaacatccagcggtttctgcccaatcctgctggcgtgcagctggaagatcctgagttccaggcctccaacatcatgcactccatcaatggctatgtgttcgacagcctgcagctgagcgtgtgcctgcacgaagtggcctactggtacatcctgagcattggcgcccagaccgacttcctgtccgtgttctttagcggctacaccttcaagcacaagatggtgtacgaggataccctgacactgttcccattcagcggcgagacagtgttcatgagcatggaaaaccccggcctgtggatcctgggctgtcacaacagcgacttccggaacagaggcatgacagccctgctgaaggtgtccagctgcgacaagaacaccggcgactactacgaggacagctatgaggacatcagcgcctacctgctgagcaagaacaatgccatcgagccaagaagcttcagccagaatagcagacacccctccaccagacagaagcagttcaacgccacaacaatccccgagaacgacatcgagaaaaccgatccttggtttgcccacagaacccctatgcctaagatccagaacgtgtcctccagcgatctgctgatgctcctgagacagagccctacacctcacggactgagcctgtccgatctgcaagaggccaaatacgaaaccttcagcgacgacccttctcctggcgccatcgacagcaacaatagcctgagcgagatgacccacttcagaccacagctgcaccacagcggcgacatggtgtttacacctgagagcggcctccagctgagactgaatgagaagctgggaaccaccgccgccaccgagctgaagaaactggacttcaaggtgtcctctaccagcaacaacctgatcagcacaatcccctccgacaacctggctgccggcaccgacaacacatcttctctgggcccacctagcatgcccgtgcactacgatagccagctggataccacactgttcggcaagaagtctagccctctgacagagtctggcggccctctgtctctgagcgaggaaaacaacgacagcaagctgacccgcgagatcaccagaaccacactgcagagcgaccaagaggaaatcgattacgacgacaccatcagcgtcgagatgaagaaagaagatttcgacatctacgacgaggacgagaatcagagccccagaagctttcagaaaaagacccggcactacttcattgccgccgtcgagagactgtgggactacggcatgtctagcagccctcacgtgctgagaaatagagcccagagcggcagcgtgccccagttcaagaaagtggtgttccaagagttcaccgacggcagcttcacccagccactgtatagaggcgagctgaacgagcatctgggcctgctgggcccttatatcagagccgaagtggaagataacatcatggtcaccttccggaatcaggcctctcggccctacagcttctacagctccctgatctcctacgaagaggaccagagacagggcgctgagcccagaaagaacttcgtgaagcccaacgagactaagacctacttttggaaggtgcagcaccacatggcccctacaaaggacgagttcgactgcaaggcctgggcctacttttccgatgtggatctggaaaaggacgtgcacagcgggctcatcggaccactgcttgtgtgccacaccaacacactgaaccccgctcacggcagacaagtgacagtgcaagagttcgccctgttcttcaccatcttcgacgaaacaaagagctggtacttcaccgagaatatggaacggaactgtcgggccccttgcaacatccagatggaagatcccaccttcaaagagaactaccggttccacgccatcaacggctacatcatggacacactgcccggcctggttatggctcaggatcagagaatccggtggtatctgctgtccatgggctccaacgagaatatccacagcatccacttcagcggccacgtgttcaccgtgcggaaaaaagaagagtacaaaatggccctgtacaatctgtaccctggggtgttcgaaaccgtggaaatgctgccttccaaggccggcatttggagagtggaatgtctgattggagagcacctccacgccggaatgagcaccctgtttctggtgtactccaacaagtgtcagacccctctcggcatggcctctggacacatcagagacttccagatcaccgcctctggccagtacggacagtgggctcctaaactggctcggctgcactactccggcagcatcaatgcctggtccaccaaagagcccttcagctggatcaaggtggacctgctggctcccatgatcatccacggaatcaagacccagggcgcaagacagaagttcagcagcctgtacatcagccagttcatcatcatgtacagcctggacggaaagaagtggcagacctaccggggcaatagcaccggcacactcatggtgttcttcggcaacgtggactccagcggcattaagcacaacatcttcaaccctccaatcattgcccggtacatccggctgcaccccacacactacagcatccggtctaccctgagaatggaactgatgggctgcgacctgaacagctgcagcatgcccctcggaatggaaagcaaggccatcagcgacgcccagatcacagccagcagctacttcaccaacatgttcgccacttggagcccctccaaggctagactgcatctgcagggcagaagcaacgcttggaggccccaagtgaacaaccccaaagagtggctgcaggtcgactttcaaaagaccatgaaagtgaccggcgtgaccacacagggcgtcaagtctctgctgacctctatgtacgtgaaagagttcctgattagcagcagccaggacggccaccagtggaccctgtttttccagaacggcaaagtgaaagtgttccagggcaatcaggacagcttcacacccgtggtcaactccctggatcctccactgctgaccagatacctgcggattcaccctcagtcttgggtgcaccagatcgctctgcggatggaagtgctgggctgtgaagctcaggacctctactga

SEQ ID NO: 8 - DNA, 5013 bp, synthetic construct
  source 1..5013: mol_type = other DNA
atgcagattgagctcagcacatgcttctttctctgtctgctgaggttctgcttcagcgccacaagaaggtactatctcggagctgtggaactgagctgggactatatgcaaagcgatctgggcgaactgcccgtggatgccagattcccccccagagtgcctaagtccttccctttcaacaccagcgtggtctataagaagacactgttcgtcgagttcacagaccatctgttcaacatcgctaagcctaggcctccttggatgggactgctgggccccaccatccaagccgaggtgtacgataccgtggtgatcacactcaaaaacatggcctcccaccccgtgtccctccatgctgtgggagtctcctactggaaggcttccgaaggagccgagtatgacgatcagaccagccaaagggagaaagaagacgacaaagtgttccccggcggatcccatacctacgtctggcaagtgctcaaagagaatggccccatggctagcgatcccctctgcctcacatattcctatctgagccatgtggatctcgtcaaggatctgaactccggactgattggagctctgctggtctgtagggaaggatctctggctaaagagaaaacccagaccctccacaagttcattctgctcttcgccgtgttcgacgagggaaaaagctggcacagcgagacaaagaacagcctcatgcaagacagagatgctgcttccgccagagcttggcccaagatgcacaccgtcaacggctacgtgaataggagcctccccggcctcattggctgccacagaaagtccgtgtactggcacgtgattggcatgggaaccacccccgaggtgcactccatcttcctcgagggacacacatttctcgtgaggaaccacagacaagccagcctcgagatcagccccattacctttctgaccgctcagacactgctcatggacctcggacaatttctgctgttctgccacatcagctcccaccagcacgatggcatggaggcttatgtcaaggtcgatagctgccccgaggaacctcagctgagaatgaagaacaatgaagaggccgaggactacgacgacgatctgaccgatagcgagatggatgtcgtgagattcgacgacgacaacagccctagctttatccagattaggagcgtggccaagaaacaccccaaaacatgggtgcactacattgccgctgaggaagaggactgggattatgctcctctggtgctcgcccccgacgataggagctacaagtcccaatatctgaacaacggccctcaaaggatcggaagaaaatacaaaaaggtgagattcatggcttacaccgacgagacctttaagacaagggaggccatccagcatgaatccggaattctgggacctctgctctacggagaggtgggagacacactgctcattatcttcaagaatcaagcctctaggccctacaacatctatcctcacggcattacagacgtcagacctctgtattccagaaggctccccaagggcgtcaaacatctcaaggactttcccattctgcccggcgaaatcttcaaatacaagtggacagtgaccgtcgaagatggccctaccaaatccgaccctaggtgtctgacaaggtactattcctcctttgtgaacatggagagggatctggccagcggcctcatcggccctctcctcatctgctataaagagagcgtcgatcagagaggcaatcagatcatgtccgacaaaaggaacgtcatcctcttctccgtcttcgacgagaatagaagctggtatctgaccgagaacatccagagattcctccctaaccccgccggcgtccagctggaggatcccgagtttcaagcctccaatatcatgcactccattaatggctacgtgttcgactctctgcagctctccgtctgtctgcatgaggtggcttattggtacattctgagcatcggcgctcagacagattttctgtccgtcttcttcagcggctatacattcaagcataagatggtctatgaggacaccctcacactgttccccttctccggcgagaccgtcttcatgagcatggaaaaccccggactctggattctcggctgccacaattccgatttcagaaataggggaatgaccgctctgctgaaggtgagcagctgtgacaagaacaccggcgattattatgaggacagctacgaggacatttccgcctatctgctctccaagaacaacgctatcgagcctaggagcttctcccaaaattctaggcacccttccacaaggcagaagcaatttaacgccaccaccatccccgagaacgacattgagaagacagacccttggttcgcccataggacacccatgcccaagattcagaacgtcagcagctccgatctgctcatgctgctcagacaatcccctacaccccatggactctctctgtccgatctccaagaggccaaatacgagaccttctccgatgacccctcccccggcgccattgattccaacaactccctctccgaaatgacccactttagaccccaactgcaccactccggcgacatggtctttacccccgaatccggactgcagctgaggctgaacgagaagctgggcaccacagccgccacagaactcaaaaaactggattttaaagtgtcctccaccagcaacaatctgatcagcaccatcccctccgacaacctcgccgctggaacagacaacacctccagcctcggacccccttccatgcccgtgcactatgattcccagctcgacaccacactcttcggaaaaaagtcctcccctctcaccgaaagcggcggacctctgtctctgagcgaggaaaacaacgactccaagctgctggaatccggactgatgaatagccaagagagcagctggggcaagaacgtgagcagcagggagatcacaagaacaacactgcagtccgaccaagaggaaattgactacgatgataccattagcgtggagatgaagaaggaagacttcgatatttacgacgaagatgagaatcagagccctaggtccttccagaagaaaaccagacactacttcatcgccgctgtcgaaaggctctgggactacggcatgtcctccagcccccatgtgctgaggaatagggctcagagcggctccgtgccccagttcaagaaggtcgtctttcaagagtttaccgacggaagctttacccagcctctgtataggggagagctcaacgagcatctgggactgctcggcccttatattagagccgaagtggaagataatatcatggtgacatttaggaaccaagcctctaggccttatagcttctacagctccctcatcagctatgaggaagaccaaagacaaggcgccgagcctaggaagaactttgtcaagcccaacgagaccaagacctacttttggaaggtgcagcatcacatggctcctaccaaggacgaatttgattgtaaggcttgggcctacttcagcgacgtcgatctggaaaaggacgtgcattccggactgatcggacccctcctcgtctgtcataccaatacactgaaccccgcccacggaaggcaagtgaccgtccaagagttcgctctgttcttcaccattttcgatgaaaccaagagctggtactttacagaaaacatggaaaggaattgtagggccccttgcaacattcaaatggaagatcctacctttaaggagaattataggtttcacgccatcaacggctatatcatggataccctccccggactggtcatggcccaagaccagaggattaggtggtatctgctgagcatgggatccaacgaaaacatccacagcatccatttctccggacacgtctttaccgtgaggaagaaggaggagtataagatggccctctataatctctatcccggcgtgttcgaaaccgtggaaatgctgccctccaaggccggcatttggagagtggagtgtctgattggcgaacatctgcatgccggaatgagcacactctttctcgtgtacagcaacaagtgtcaaacacctctgggcatggctagcggacacatcagagacttccaaattaccgcctccggacagtacggacaatgggcccctaaactcgctaggctccactactccggatccatcaatgcttggtccaccaaggagcctttcagctggatcaaggtggatctcctcgcccccatgatcatccatggcattaagacccaaggcgctagacagaaatttagcagcctctacatctcccagtttattatcatgtactctctggatggcaagaagtggcaaacctatagaggcaacagcaccggcacactgatggtgttcttcggaaacgtggacagctccggcattaagcataacatcttcaacccccccatcattgctaggtatattaggctgcaccccacccactatagcattaggtccacactgaggatggagctgatgggctgcgatctgaacagctgcagcatgcccctcggaatggagtccaaggccatcagcgatgctcagatcaccgctagctcctacttcacaaacatgttcgccacatggtccccttccaaagctaggctgcacctccaaggcagaagcaatgcttggaggccccaagtcaacaatcccaaggagtggctgcaagtggatttccagaagaccatgaaagtcaccggcgtcacaacccaaggcgtgaaatctctgctgacatccatgtacgtgaaggagtttctgatctccagctcccaagacggccatcaatggaccctctttttccagaacggcaaggtgaaagtgttccaaggcaaccaagacagctttacacccgtggtgaatagcctcgacccccctctcctcacaaggtacctcagaattcacccccaaagctgggtccaccagattgctctgagaatggaggtcctcggctgcgaagcccaagacctctattga

SEQ ID NO: 9 - DNA, 4959 bp, synthetic construct
  source 1..4959: mol_type = other DNA
atgcagatcgagctgtctacctgcttcttcctgtgcctgctgcggttctgcttcagcgccaccagaagatattacctgggcgccgtggaactgagctgggactacatgcagtctgacctgggagagctgcccgtggacgctagatttcctccaagagtgcccaagagcttccccttcaacacctccgtggtgtacaagaaaaccctgttcgtggaattcaccgaccacctgttcaatatcgccaagcctcggcctccttggatgggactgctgggacctacaattcaggccgaggtgtacgacaccgtggtcatcaccctgaagaacatggccagccatcctgtgtctctgcacgccgtgggagtgtcttactggaaggcttctgagggcgccgagtacgacgatcagacaagccagagagagaaagaggacgacaaggttttccctggcggcagccacacctatgtctggcaggtcctgaaagaaaacggccctatggcctccgatcctctgtgcctgacatacagctacctgagccacgtggacctggtcaaggacctgaattctggcctgatcggagccctgctcgtgtgtagagaaggcagcctggccaaagagaaaacccagacactgcacaagttcatcctgctgttcgccgtgttcgacgagggcaagagctggcacagcgagacaaagaacagcctgatgcaggacagggatgccgcctctgctagagcttggcctaagatgcacaccgtgaacggctacgtgaacagaagcctgcctggactgatcggctgccacagaaagtccgtgtactggcacgtgatcggcatgggcacaacacctgaggtgcacagcatctttctggaaggacacaccttcctcgtgcggaaccatagacaggccagcctggaaatcagccctatcaccttcctgaccgctcagaccctgctgatggatctgggccagtttctgctgttctgccacatcagctcccaccagcacgatggcatggaagcctacgtgaaggtggacagctgccccgaagaaccccagctgcggatgaagaacaacgaggaagccgaggactacgacgacgacctgaccgactctgagatggacgtcgtcagattcgacgacgataacagccccagcttcatccagatcagaagcgtggccaagaagcaccccaagacctgggtgcactatatcgccgccgaggaagaggactgggattacgctcctctggtgctggcccctgacgacagaagctacaagagccagtacctgaacaacggccctcagcggatcggccggaagtataagaaagtgcggttcatggcctacaccgacgagacattcaagaccagagaggccatccagcacgagagcggaattctgggccctctgctgtatggcgaagtgggcgatacactgctgatcatcttcaagaaccaggccagcagaccctacaacatctaccctcacggcatcaccgatgtgcggcccctgtattctagaaggctgcccaagggcgtgaagcacctgaaggacttccctatcctgcctggcgagatcttcaagtacaagtggaccgtgaccgtggaagatggccccaccaagagcgaccctagatgtctgacacggtactacagcagcttcgtgaacatggaacgcgacctggccagcggcctgattggacctctgctgatctgctacaaagaaagcgtggaccagcggggcaaccagatcatgagcgacaagcggaacgtgatcctgtttagcgtgttcgatgagaaccggtcctggtatctgaccgagaacatccagcggtttctgcccaatcctgctggcgtgcagctggaagatcctgagttccaggcctccaacatcatgcactccatcaatggctatgtgttcgacagcctgcagctgagcgtgtgcctgcacgaagtggcctactggtacatcctgagcattggcgcccagaccgacttcctgtccgtgttctttagcggctacaccttcaagcacaagatggtgtacgaggataccctgacactgttcccattcagcggcgagacagtgttcatgagcatggaaaaccccggcctgtggatcctgggctgtcacaacagcgacttccggaacagaggcatgacagccctgctgaaggtgtccagctgcgacaagaacaccggcgactactacgaggacagctatgaggacatcagcgcctacctgctgagcaagaacaatgccatcgagacaagaagcttcagccagaatagcagacacccctccaccagacagaagcagttcaacgccacaacaatccccgagaacgacatcgagaaaaccgatccttggtttgcccacagaacccctatgcctaagatccagaacgtgtcctccagcgatctgctgatgctcctgagacagagccctacacctcacggactgagcctgtccgatctgcaagaggccaaatacgaaaccttcagcgacgacccttctcctggcgccatcgacagcaacaatagcctgagcgagatgacccacttcagaccacagctgcaccacagcggcgacatggtgtttacacctgagagcggcctccagctgagactgaatgagaagctgggaaccaccgccgccaccgagctgaagaaactggacttcaaggtgtcctctaccagcaacaacctgatcagcacaatcccctccgacaacctggctgccggcaccgacaacacatcttctctgggcccacctagcatgcccgtgcactacgatagccagctggataccacactgttcggcaagaagtctagccctctgacagagtctggcggccctctgtctctgagcgaggaaaacaacgacagcaagctgacccgcgagatcaccagaaccacactgcagagcgaccaagaggaaatcgattacgacgacaccatcagcgtcgagatgaagaaagaagatttcgacatctacgacgaggacgagaatcagagccccagaagctttcagaaaaagacccggcactacttcattgccgccgtcgagagactgtgggactacggcatgtctagcagccctcacgtgctgagaaatagagcccagagcggcagcgtgccccagttcaagaaagtggtgttccaagagttcaccgacggcagcttcacccagccactgtatagaggcgagctgaacgagcatctgggcctgctgggcccttatatcagagccgaagtggaagataacatcatggtcaccttccggaatcaggcctctcggccctacagcttctacagctccctgatctcctacgaagaggaccagagacagggcgctgagcccagaaagaacttcgtgaagcccaacgagactaagacctacttttggaaggtgcagcaccacatggcccctacaaaggacgagttcgactgcaaggcctgggcctacttttccgatgtggatctggaaaaggacgtgcacagcgggctcatcggaccactgcttgtgtgccacaccaacacactgaaccccgctcacggcagacaagtgacagtgcaagagttcgccctgttcttcaccatcttcgacgaaacaaagagctggtacttcaccgagaatatggaacggaactgtcgggccccttgcaacatccagatggaagatcccaccttcaaagagaactaccggttccacgccatcaacggctacatcatggacacactgcccggcctggttatggctcaggatcagagaatccggtggtatctgctgtccatgggctccaacgagaatatccacagcatccacttcagcggccacgtgttcaccgtgcggaaaaaagaagagtacaaaatggccctgtacaatctgtaccctggggtgttcgaaaccgtggaaatgctgccttccaaggccggcatttggagagtggaatgtctgattggagagcacctccacgccggaatgagcaccctgtttctggtgtactccaacaagtgtcagacccctctcggcatggcctctggacacatcagagacttccagatcaccgcctctggccagtacggacagtgggctcctaaactggctcggctgcactactccggcagcatcaatgcctggtccaccaaagagcccttcagctggatcaaggtggacctgctggctcccatgatcatccacggaatcaagacccagggcgcaagacagaagttcagcagcctgtacatcagccagttcatcatcatgtacagcctggacggaaagaagtggcagacctaccggggcaatagcaccggcacactcatggtgttcttcggcaacgtggactccagcggcattaagcacaacatcttcaaccctccaatcattgcccggtacatccggctgcaccccacacactacagcatccggtctaccctgagaatggaactgatgggctgcgacctgaacagctgcagcatgcccctcggaatggaaagcaaggccatcagcgacgcccagatcacagccagcagctacttcaccaacatgttcgccacttggagcccctccaaggctagactgcatctgcagggcagaagcaacgcttggaggccccaagtgaacaaccccaaagagtggctgcaggtcgactttcaaaagaccatgaaagtgaccggcgtgaccacacagggcgtcaagtctctgctgacctctatgtacgtgaaagagttcctgattagcagcagccaggacggccaccagtggaccctgtttttccagaacggcaaagtgaaagtgttccagggcaatcaggacagcttcacacccgtggtcaactccctggatcctccactgctgaccagatacctgcggattcaccctcagtcttgggtgcaccagatcgctctgcggatggaagtgctgggctgtgaagctcaggacctctactga

SEQ ID NO: 10 - protein, 1464 aa, synthetic construct
MQIELSTCFFLCLLRFCFSATRRYYLGAVELSWDYMQSDLGELPVDARFPPRVPKSFPFNTSVVYKKTLFVEFTDHLFNIAKPRPPWMGLLGPTIQAEVYDTVVITLKNMASHPVSLHAVGVSYWKASEGAEYDDQTSQREKEDDKVFPGGSHTYVWQVLKENGPMASDPLCLTYSYLSHVDLVKDLNSGLIGALLVCREGSLAKEKTQTLHKFILLFAVFDEGKSWHSETKNSLMQDRDAASARAWPKMHTVNGYVNRSLPGLIGCHRKSVYWHVIGMGTTPEVHSIFLEGHTFLVRNHRQASLEISPITFLTAQTLLMDLGQFLLFCHISSHQHDGMEAYVKVDSCPEEPQLRMKNNEEAEDYDDDLTDSEMDVVRFDDDNSPSFIQIRSVAKKHPKTWVHYIAAEEEDWDYAPLVLAPDDRSYKSQYLNNGPQRIGRKYKKVRFMAYTDETFKTREAIQHESGILGPLLYGEVGDTLLIIFKNQASRPYNIYPHGITDVRPLYSRRLPKGVKHLKDFPILPGEIFKYKWTVTVEDGPTKSDPRCLTRYYSSFVNMERDLASGLIGPLLICYKESVDQRGNQIMSDKRNVILFSVFDENRSWYLTENIQRFLPNPAGVQLEDPEFQASNIMHSINGYVFDSLQLSVCLHEVAYWYILSIGAQTDFLSVFFSGYTFKHKMVYEDTLTLFPFSGETVFMSMENPGLWILGCHNSDFRNRGMTALLKVSSCDKNTGDYYEDSYEDISAYLLSKNNAIEPRSFSQNSRHPSQNPPVLKRHQREITRTTLQSDQEEIDYDDTISVEMKKEDFDIYDEDENQSPRSFQKKTRHYFIAAVERLWDYGMSSSPHVLRNRAQSGSVPQFKKVVFQEFTDGSFTQPLYRGELNEHLGLLGPYIRAEVEDNIMVTFRNQASRPYSFYSSLISYEEDQRQGAEPRKNFVKPNETKTYFWKVQHHMAPTKDEFDCKAWAYFSDVDLEKDVHSGLIGPLLVCHTNTLNPAHGRQVTVQEFALFFTIFDETKSWYFTENMERNCRAPCNIQMEDPTFKENYRFHAINGYIMDTLPGLVMAQDQRIRWYLLSMGSNENIHSIHFSGHVFTVRKKEEYKMALYNLYPGVFETVEMLPSKAGIWRVECLIGEHLHAGMSTLFLVYSNKCQTPLGMASGHIRDFQITASGQYGQWAPKLARLHYSGSINAWSTKEPFSWIKVDLLAPMIIHGIKTQGARQKFSSLYISQFIIMYSLDGKKWQTYRGNSTGTLMVFFGNVDSSGIKHNIFNPPIIARYIRLHPTHYSIRSTLRMELMGCDLNSCSMPLGMESKAISDAQITASSYFTNMFATWSPSKARLHLQGRSNAWRPQVNNPKEWLQVDFQKTMKVTGVTTQGVKSLLTSMYVKEFLISSSQDGHQWTLFFQNGKVKVFQGNQDSFTPVVNSLDPPLLTRYLRIHPQSWVHQIALRMEVLGCEAQDLY

SEQ ID NO: 11 - DNA, 4395 bp, synthetic construct
  source 1..4395: mol_type = other DNA
atgcagatcgagctgtctacctgcttcttcctgtgcctgctgcggttctgcttcagcgccaccagacggtactatctgggcgccgtggaactgagctgggactacatgcagagcgacctgggcgagctgcccgtggatgccagattccctccaagagtgcccaagagcttccccttcaacacctccgtggtgtacaagaaaaccctgttcgtggaattcaccgaccacctgttcaatatcgccaagcccagacccccctggatgggcctgctgggacctacaattcaggccgaggtgtacgacaccgtcgtgatcaccctgaagaacatggccagccaccccgtgtctctgcatgccgtgggagtgtcctactggaaggcctctgagggcgccgagtacgacgatcagaccagccagcgcgagaaagaggacgacaaggtgttccctggcggcagccacacctacgtgtggcaggtgctgaaagaaaacggccccatggcctccgaccctctgtgcctgacatacagctacctgagccacgtggacctcgtgaaggacctgaacagcggcctgatcggagccctgctcgtgtgtagagagggcagcctggccaaagagaaaacccagaccctgcacaagttcatcctgctgttcgccgtgttcgacgagggcaagagctggcacagcgagacaaagaacagcctgatgcaggaccgggacgccgcctctgctagagcctggcccaaaatgcacaccgtgaacggctacgtgaacagaagcctgcccggactgatcggctgccaccggaagtctgtgtactggcacgtgatcggcatgggcaccacccctgaggtgcacagcatctttctggaaggacacacctttctcgtgcggaaccaccggcaggccagcctggaaatcagccctatcaccttcctgaccgcccagacactgctgatggacctgggccagtttctgctgttctgccacatcagctcccaccagcacgacggcatggaagcctacgtgaaggtggacagctgccccgaggaaccccagctgcggatgaagaacaacgaggaagccgaggactacgacgacgacctgaccgacagcgagatggacgtggtgcgcttcgacgacgataacagccccagcttcatccagatcagaagcgtggccaagaagcaccccaagacctgggtgcactatatcgccgccgaggaagaggactgggattacgcccctctggtgctggcccccgacgacagaagctacaagagccagtacctgaacaatggcccccagcggatcggccggaagtataagaaagtgcggttcatggcctacaccgacgagacattcaagaccagagaggccatccagcacgagagcggcatcctgggccctctgctgtatggcgaagtgggcgacaccctgctgatcatcttcaagaaccaggccagcagaccctacaacatctaccctcacggcatcaccgacgtgcggcccctgtactctagaaggctgcccaagggcgtgaaacacctgaaggacttccccatcctgcccggcgagatcttcaagtacaagtggaccgtgaccgtggaagatggccccaccaagagcgaccccagatgcctgacacggtactacagcagcttcgtgaacatggaacgggacctggcctccggcctgattggcccactgctgatctgctacaaagaaagcgtggaccagcggggcaaccagatcatgagcgacaagcggaacgtgatcctgtttagcgtgttcgatgagaaccggtcctggtatctgaccgagaatatccagcggttcctgcccaaccctgccggcgtgcagctggaagatcctgagttccaggcctccaacatcatgcactccatcaatggctatgtgttcgacagcctgcagctgagcgtgtgcctgcacgaggtggcctactggtacatcctgagcatcggggcccagaccgacttcctgtccgtgttcttctccggctacaccttcaagcacaagatggtgtacgaggataccctgaccctgttcccctttagcggcgaaaccgtgttcatgagcatggaaaaccccggcctgtggatcctgggctgccacaacagcgacttccggaacagaggcatgaccgccctgctgaaggtgtccagctgcgacaagaacaccggcgactactacgaggacagctatgaggacatcagcgcctacctgctgagcaagaacaatgccatcgagcccagaagcttcagccagaactcccggcaccctagccagaaccctcccgtgctgaagcggcaccagagagagatcacccggaccaccctgcagtccgaccaggaagagatcgattacgacgacaccatcagcgtggaaatgaagaaagaagatttcgacatctacgacgaggacgagaaccagagcccccggtcctttcagaaaaagacccggcactacttcattgccgctgtggaacggctgtgggactacggcatgagcagcagcccacacgtgctgagaaacagggcccagagcggcagcgtgccccagttcaagaaagtggtgttccaggaattcacagacggcagcttcacccagcctctgtaccgcggcgagctgaatgagcacctgggactgctgggcccctatatcagagccgaagtggaagataacatcatggtcaccttccggaatcaggcctcccggccctacagcttctacagctccctgatcagctacgaagaggaccagagacagggcgctgagccccggaagaacttcgtgaagcccaacgagactaagacctacttttggaaggtgcagcaccacatggcccctacaaaggacgagttcgactgcaaggcctgggcctacttctccgatgtggacctggaaaaggacgtgcactctgggctgatcggccccctgctcgtgtgccacaccaacaccctgaatcccgcccacggcagacaagtgacagtgcaggaattcgccctgttcttcaccatcttcgacgaaacaaagagctggtacttcaccgaaaacatggaaagaaactgccgggctccctgcaacatccagatggaagatcccaccttcaaagagaactaccggttccacgccatcaacggctacatcatggacacactgcccggcctcgtgatggctcaggatcagcggatccggtggtatctgctgtccatgggctccaacgagaacatccacagcatccacttcagcggccacgtgttcaccgtgcggaaaaaagaagagtacaaaatggccctgtacaacctgtaccctggggtgttcgagacagtggaaatgctgcccagcaaggccggcatctggcgggtggaatgtctgatcggcgagcatctgcacgctgggatgagcacactgtttctggtgtacagcaacaagtgccagacacctctgggcatggcctctggccacatccgggactttcagatcacagccagcggccagtatggccagtgggccccaaaactggccagactgcactacagcggcagcatcaacgcctggtccaccaaagagcccttcagctggatcaaggtggacctgctggctcccatgatcatccacggaatcaagacccagggcgccagacagaagttcagcagcctgtacatcagccagttcatcatcatgtacagcctggacggcaagaagtggcagacctaccggggcaatagcaccggcacactgatggtgttcttcggcaacgtggactccagcggcattaagcacaacatcttcaacccccccatcattgcccggtacatccggctgcaccccacccactacagcatccggtccaccctgagaatggaactgatgggctgcgacctgaactcctgcagcatgcccctggggatggaaagcaaggccatctccgacgcccagatcaccgcctccagctacttcaccaacatgttcgccacctggtccccatccaaggcccggctgcatctgcagggcagaagcaatgcttggaggccccaagtgaacaaccccaaagaatggctgcaggtggacttccagaaaaccatgaaagtgaccggcgtgaccacccagggcgtgaagtctctgctgacctctatgtacgtgaaagagttcctgatctccagcagccaggacggccaccagtggaccctgtttttccagaacggcaaagtgaaagtgtttcaggggaaccaggactccttcacccccgtcgtgaatagcctggatcccccactgctgaccagatacctgcggatccaccctcagagttgggtgcaccagattgctctgcggatggaagtgctgggatgcgaggcccaggacctgtactga

SEQ ID NO: 12 - protein, 1680 aa, synthetic construct
MQIELSTCFFLCLLRFCFSATRRYYLGAVELSWDYMQSDLGELPVDARFPPRVPKSFPFNTSVVYKKTLFVEFTDHLFNIAKPRPPWMGLLGPTIQAEVYDTVVITLKNMASHPVSLHAVGVSYWKASEGAEYDDQTSQREKEDDKVFPGGSHTYVWQVLKENGPMASDPLCLTYSYLSHVDLVKDLNSGLIGALLVCREGSLAKEKTQTLHKFILLFAVFDEGKSWHSETKNSLMQDRDAASARAWPKMHTVNGYVNRSLPGLIGCHRKSVYWHVIGMGTTPEVHSIFLEGHTFLVRNHRQASLEISPITFLTAQTLLMDLGQFLLFCHISSHQHDGMEAYVKVDSCPEEPQLRMKNNEEAEDYDDDLTDSEMDVVRFDDDNSPSFIQIRSVAKKHPKTWVHYIAAEEEDWDYAPLVLAPDDRSYKSQYLNNGPQRIGRKYKKVRFMAYTDETFKTREAIQHESGILGPLLYGEVGDTLLIIFKNQASRPYNIYPHGITDVRPLYSRRLPKGVKHLKDFPILPGEIFKYKWTVTVEDGPTKSDPRCLTRYYSSFVNMERDLASGLIGPLLICYKESVDQRGNQIMSDKRNVILFSVFDENRSWYLTENIQRFLPNPAGVQLEDPEFQASNIMHSINGYVFDSLQLSVCLHEVAYWYILSIGAQTDFLSVFFSGYTFKHKMVYEDTLTLFPFSGETVFMSMENPGLWILGCHNSDFRNRGMTALLKVSSCDKNTGDYYEDSYEDISAYLLSKNNAIEPRSFSQNSRHPSTRQKQFNATTIPENDIEKTDPWFAHRTPMPKIQNVSSSDLLMLLRQSPTPHGLSLSDLQEAKYETFSDDPSPGAIDSNNSLSEMTHFRPQLHHSGDMVFTPESGLQLRLNEKLGTTAATELKKLDFKVSSTSNNLISTIPSDNLAAGTDNTSSLGPPSMPVHYDSQLDTTLFGKKSSPLTESGGPLSLSEENNDSKLLESGLMNSQESSWGKNVSSQNPPVLKRHQREITRTTLQSDQEEIDYDDTISVEMKKEDFDIYDEDENQSPRSFQKKTRHYFIAAVERLWDYGMSSSPHVLRNRAQSGSVPQFKKVVFQEFTDGSFTQPLYRGELNEHLGLLGPYIRAEVEDNIMVTFRNQASRPYSFYSSLISYEEDQRQGAEPRKNFVKPNETKTYFWKVQHHMAPTKDEFDCKAWAYFSDVDLEKDVHSGLIGPLLVCHTNTLNPAHGRQVTVQEFALFFTIFDETKSWYFTENMERNCRAPCNIQMEDPTFKENYRFHAINGYIMDTLPGLVMAQDQRIRWYLLSMGSNENIHSIHFSGHVFTVRKKEEYKMALYNLYPGVFETVEMLPSKAGIWRVECLIGEHLHAGMSTLFLVYSNKCQTPLGMASGHIRDFQITASGQYGQWAPKLARLHYSGSINAWSTKEPFSWIKVDLLAPMIIHGIKTQGARQKFSSLYISQFIIMYSLDGKKWQTYRGNSTGTLMVFFGNVDSSGIKHNIFNPPIIARYIRLHPTHYSIRSTLRMELMGCDLNSCSMPLGMESKAISDAQITASSYFTNMFATWSPSKARLHLQGRSNAWRPQVNNPKEWLQVDFQKTMKVTGVTTQGVKSLLTSMYVKEFLISSSQDGHQWTLFFQNGKVKVFQGNQDSFTPVVNSLDPPLLTRYLRIHPQSWVHQIALRMEVLGCEAQDLY

SEQ ID NO: 13 - DNA, 5043 bp, synthetic construct
  source 1..5043: mol_type = other DNA
atgcagattgagctcagcacatgcttctttctctgtctgctgaggttctgcttcagcgccacaagaaggtactatctcggagctgtggaactgagctgggactatatgcaaagcgatctgggcgaactgcccgtggatgccagattcccccccagagtgcctaagtccttccctttcaacaccagcgtggtctataagaagacactgttcgtcgagttcacagaccatctgttcaacatcgctaagcctaggcctccttggatgggactgctgggccccaccatccaagccgaggtgtacgataccgtggtgatcacactcaaaaacatggcctcccaccccgtgtccctccatgctgtgggagtctcctactggaaggcttccgaaggagccgagtatgacgatcagaccagccaaagggagaaagaagacgacaaagtgttccccggcggatcccatacctacgtctggcaagtgctcaaagagaatggccccatggctagcgatcccctctgcctcacatattcctatctgagccatgtggatctcgtcaaggatctgaactccggactgattggagctctgctggtctgtagggaaggatctctggctaaagagaaaacccagaccctccacaagttcattctgctcttcgccgtgttcgacgagggaaaaagctggcacagcgagacaaagaacagcctcatgcaagacagagatgctgcttccgccagagcttggcccaagatgcacaccgtcaacggctacgtgaataggagcctccccggcctcattggctgccacagaaagtccgtgtactggcacgtgattggcatgggaaccacccccgaggtgcactccatcttcctcgagggacacacatttctcgtgaggaaccacagacaagccagcctcgagatcagccccattacctttctgaccgctcagacactgctcatggacctcggacaatttctgctgttctgccacatcagctcccaccagcacgatggcatggaggcttatgtcaaggtcgatagctgccccgaggaacctcagctgagaatgaagaacaatgaagaggccgaggactacgacgacgatctgaccgatagcgagatggatgtcgtgagattcgacgacgacaacagccctagctttatccagattaggagcgtggccaagaaacaccccaaaacatgggtgcactacattgccgctgaggaagaggactgggattatgctcctctggtgctcgcccccgacgataggagctacaagtcccaatatctgaacaacggccctcaaaggatcggaagaaaatacaaaaaggtgagattcatggcttacaccgacgagacctttaagacaagggaggccatccagcatgaatccggaattctgggacctctgctctacggagaggtgggagacacactgctcattatcttcaagaatcaagcctctaggccctacaacatctatcctcacggcattacagacgtcagacctctgtattccagaaggctccccaagggcgtcaaacatctcaaggactttcccattctgcccggcgaaatcttcaaatacaagtggacagtgaccgtcgaagatggccctaccaaatccgaccctaggtgtctgacaaggtactattcctcctttgtgaacatggagagggatctggccagcggcctcatcggccctctcctcatctgctataaagagagcgtcgatcagagaggcaatcagatcatgtccgacaaaaggaacgtcatcctcttctccgtcttcgacgagaatagaagctggtatctgaccgagaacatccagagattcctccctaaccccgccggcgtccagctggaggatcccgagtttcaagcctccaatatcatgcactccattaatggctacgtgttcgactctctgcagctctccgtctgtctgcatgaggtggcttattggtacattctgagcatcggcgctcagacagattttctgtccgtcttcttcagcggctatacattcaagcataagatggtctatgaggacaccctcacactgttccccttctccggcgagaccgtcttcatgagcatggaaaaccccggactctggattctcggctgccacaattccgatttcagaaataggggaatgaccgctctgctgaaggtgagcagctgtgacaagaacaccggcgattattatgaggacagctacgaggacatttccgcctatctgctctccaagaacaacgctatcgagcctaggagcttctcccaaaattctaggcacccttccacaaggcagaagcaatttaacgccaccaccatccccgagaacgacattgagaagacagacccttggttcgcccataggacacccatgcccaagattcagaacgtcagcagctccgatctgctcatgctgctcagacaatcccctacaccccatggactctctctgtccgatctccaagaggccaaatacgagaccttctccgatgacccctcccccggcgccattgattccaacaactccctctccgaaatgacccactttagaccccaactgcaccactccggcgacatggtctttacccccgaatccggactgcagctgaggctgaacgagaagctgggcaccacagccgccacagaactcaaaaaactggattttaaagtgtcctccaccagcaacaatctgatcagcaccatcccctccgacaacctcgccgctggaacagacaacacctccagcctcggacccccttccatgcccgtgcactatgattcccagctcgacaccacactcttcggaaaaaagtcctcccctctcaccgaaagcggcggacctctgtctctgagcgaggaaaacaacgactccaagctgctggaatccggactgatgaatagccaagagagcagctggggcaagaacgtgagcagccagaaccctcccgtgctgaaaaggcaccagagggagatcacaagaacaacactgcagtccgaccaagaggaaattgactacgatgataccattagcgtggagatgaagaaggaagacttcgatatttacgacgaagatgagaatcagagccctaggtccttccagaagaaaaccagacactacttcatcgccgctgtcgaaaggctctgggactacggcatgtcctccagcccccatgtgctgaggaatagggctcagagcggctccgtgccccagttcaagaaggtcgtctttcaagagtttaccgacggaagctttacccagcctctgtataggggagagctcaacgagcatctgggactgctcggcccttatattagagccgaagtggaagataatatcatggtgacatttaggaaccaagcctctaggccttatagcttctacagctccctcatcagctatgaggaagaccaaagacaaggcgccgagcctaggaagaactttgtcaagcccaacgagaccaagacctacttttggaaggtgcagcatcacatggctcctaccaaggacgaatttgattgtaaggcttgggcctacttcagcgacgtcgatctggaaaaggacgtgcattccggactgatcggacccctcctcgtctgtcataccaatacactgaaccccgcccacggaaggcaagtgaccgtccaagagttcgctctgttcttcaccattttcgatgaaaccaagagctggtactttacagaaaacatggaaaggaattgtagggccccttgcaacattcaaatggaagatcctacctttaaggagaattataggtttcacgccatcaacggctatatcatggataccctccccggactggtcatggcccaagaccagaggattaggtggtatctgctgagcatgggatccaacgaaaacatccacagcatccatttctccggacacgtctttaccgtgaggaagaaggaggagtataagatggccctctataatctctatcccggcgtgttcgaaaccgtggaaatgctgccctccaaggccggcatttggagagtggagtgtctgattggcgaacatctgcatgccggaatgagcacactctttctcgtgtacagcaacaagtgtcaaacacctctgggcatggctagcggacacatcagagacttccaaattaccgcctccggacagtacggacaatgggcccctaaactcgctaggctccactactccggatccatcaatgcttggtccaccaaggagcctttcagctggatcaaggtggatctcctcgcccccatgatcatccatggcattaagacccaaggcgctagacagaaatttagcagcctctacatctcccagtttattatcatgtactctctggatggcaagaagtggcaaacctatagaggcaacagcaccggcacactgatggtgttcttcggaaacgtggacagctccggcattaagcataacatcttcaacccccccatcattgctaggtatattaggctgcaccccacccactatagcattaggtccacactgaggatggagctgatgggctgcgatctgaacagctgcagcatgcccctcggaatggagtccaaggccatcagcgatgctcagatcaccgctagctcctacttcacaaacatgttcgccacatggtccccttccaaagctaggctgcacctccaaggcagaagcaatgcttggaggccccaagtcaacaatcccaaggagtggctgcaagtggatttccagaagaccatgaaagtcaccggcgtcacaacccaaggcgtgaaatctctgctgacatccatgtacgtgaaggagtttctgatctccagctcccaagacggccatcaatggaccctctttttccagaacggcaaggtgaaagtgttccaaggcaaccaagacagctttacacccgtggtgaatagcctcgacccccctctcctcacaaggtacctcagaattcacccccaaagctgggtccaccagattgctctgagaatggaggtcctcggctgcgaagcccaagacctctattga

SEQ ID NO: 14 - protein, 1652 aa, synthetic construct
MQIELSTCFFLCLLRFCFSATRRYYLGAVELSWDYMQSDLGELPVDARFPPRVPKSFPFNTSVVYKKTLFVEFTDHLFNIAKPRPPWMGLLGPTIQAEVYDTVVITLKNMASHPVSLHAVGVSYWKASEGAEYDDQTSQREKEDDKVFPGGSHTYVWQVLKENGPMASDPLCLTYSYLSHVDLVKDLNSGLIGALLVCREGSLAKEKTQTLHKFILLFAVFDEGKSWHSETKNSLMQDRDAASARAWPKMHTVNGYVNRSLPGLIGCHRKSVYWHVIGMGTTPEVHSIFLEGHTFLVRNHRQASLEISPITFLTAQTLLMDLGQFLLFCHISSHQHDGMEAYVKVDSCPEEPQLRMKNNEEAEDYDDDLTDSEMDVVRFDDDNSPSFIQIRSVAKKHPKTWVHYIAAEEEDWDYAPLVLAPDDRSYKSQYLNNGPQRIGRKYKKVRFMAYTDETFKTREAIQHESGILGPLLYGEVGDTLLIIFKNQASRPYNIYPHGITDVRPLYSRRLPKGVKHLKDFPILPGEIFKYKWTVTVEDGPTKSDPRCLTRYYSSFVNMERDLASGLIGPLLICYKESVDQRGNQIMSDKRNVILFSVFDENRSWYLTENIQRFLPNPAGVQLEDPEFQASNIMHSINGYVFDSLQLSVCLHEVAYWYILSIGAQTDFLSVFFSGYTFKHKMVYEDTLTLFPFSGETVFMSMENPGLWILGCHNSDFRNRGMTALLKVSSCDKNTGDYYEDSYEDISAYLLSKNNAIESRSFSQNSRHPSTRQKQFNATTIPENDIEKTDPWFAHRTPMPKIQNVSSSDLLMLLRQSPTPHGLSLSDLQEAKYETFSDDPSPGAIDSNNSLSEMTHFRPQLHHSGDMVFTPESGLQLRLNEKLGTTAATELKKLDFKVSSTSNNLISTIPSDNLAAGTDNTSSLGPPSMPVHYDSQLDTTLFGKKSSPLTESGGPLSLSEENNDSKLTREITRTTLQSDQEEIDYDDTISVEMKKEDFDIYDEDENQSPRSFQKKTRHYFIAAVERLWDYGMSSSPHVLRNRAQSGSVPQFKKVVFQEFTDGSFTQPLYRGELNEHLGLLGPYIRAEVEDNIMVTFRNQASRPYSFYSSLISYEEDQRQGAEPRKNFVKPNETKTYFWKVQHHMAPTKDEFDCKAWAYFSDVDLEKDVHSGLIGPLLVCHTNTLNPAHGRQVTVQEFALFFTIFDETKSWYFTENMERNCRAPCNIQMEDPTFKENYRFHAINGYIMDTLPGLVMAQDQRIRWYLLSMGSNENIHSIHFSGHVFTVRKKEEYKMALYNLYPGVFETVEMLPSKAGIWRVECLIGEHLHAGMSTLFLVYSNKCQTPLGMASGHIRDFQITASGQYGQWAPKLARLHYSGSINAWSTKEPFSWIKVDLLAPMIIHGIKTQGARQKFSSLYISQFIIMYSLDGKKWQTYRGNSTGTLMVFFGNVDSSGIKHNIFNPPIIARYIRLHPTHYSIRSTLRMELMGCDLNSCSMPLGMESKAISDAQITASSYFTNMFATWSPSKARLHLQGRSNAWRPQVNNPKEWLQVDFQKTMKVTGVTTQGVKSLLTSMYVKEFLISSSQDGHQWTLFFQNGKVKVFQGNQDSFTPVVNSLDPPLLTRYLRIHPQSWVHQIALRMEVLGCEAQDLY

SEQ ID NO: 15 - protein, 1652 aa, synthetic construct
MQIELSTCFFLCLLRFCFSATRRYYLGAVELSWDYMQSDLGELPVDARFPPRVPKSFPFNTSVVYKKTLFVEFTDHLFNIAKPRPPWMGLLGPTIQAEVYDTVVITLKNMASHPVSLHAVGVSYWKASEGAEYDDQTSQREKEDDKVFPGGSHTYVWQVLKENGPMASDPLCLTYSYLSHVDLVKDLNSGLIGALLVCREGSLAKEKTQTLHKFILLFAVFDEGKSWHSETKNSLMQDRDAASARAWPKMHTVNGYVNRSLPGLIGCHRKSVYWHVIGMGTTPEVHSIFLEGHTFLVRNHRQASLEISPITFLTAQTLLMDLGQFLLFCHISSHQHDGMEAYVKVDSCPEEPQLRMKNNEEAEDYDDDLTDSEMDVVRFDDDNSPSFIQIRSVAKKHPKTWVHYIAAEEEDWDYAPLVLAPDDRSYKSQYLNNGPQRIGRKYKKVRFMAYTDETFKTREAIQHESGILGPLLYGEVGDTLLIIFKNQASRPYNIYPHGITDVRPLYSRRLPKGVKHLKDFPILPGEIFKYKWTVTVEDGPTKSDPRCLTRYYSSFVNMERDLASGLIGPLLICYKESVDQRGNQIMSDKRNVILFSVFDENRSWYLTENIQRFLPNPAGVQLEDPEFQASNIMHSINGYVFDSLQLSVCLHEVAYWYILSIGAQTDFLSVFFSGYTFKHKMVYEDTLTLFPFSGETVFMSMENPGLWILGCHNSDFRNRGMTALLKVSSCDKNTGDYYEDSYEDISAYLLSKNNAIENRSFSQNSRHPSTRQKQFNATTIPENDIEKTDPWFAHRTPMPKIQNVSSSDLLMLLRQSPTPHGLSLSDLQEAKYETFSDDPSPGAIDSNNSLSEMTHFRPQLHHSGDMVFTPESGLQLRLNEKLGTTAATELKKLDFKVSSTSNNLISTIPSDNLAAGTDNTSSLGPPSMPVHYDSQLDTTLFGKKSSPLTESGGPLSLSEENNDSKLTREITRTTLQSDQEEIDYDDTISVEMKKEDFDIYDEDENQSPRSFQKKTRHYFIAAVERLWDYGMSSSPHVLRNRAQSGSVPQFKKVVFQEFTDGSFTQPLYRGELNEHLGLLGPYIRAEVEDNIMVTFRNQASRPYSFYSSLISYEEDQRQGAEPRKNFVKPNETKTYFWKVQHHMAPTKDEFDCKAWAYFSDVDLEKDVHSGLIGPLLVCHTNTLNPAHGRQVTVQEFALFFTIFDETKSWYFTENMERNCRAPCNIQMEDPTFKENYRFHAINGYIMDTLPGLVMAQDQRIRWYLLSMGSNENIHSIHFSGHVFTVRKKEEYKMALYNLYPGVFETVEMLPSKAGIWRVECLIGEHLHAGMSTLFLVYSNKCQTPLGMASGHIRDFQITASGQYGQWAPKLARLHYSGSINAWSTKEPFSWIKVDLLAPMIIHGIKTQGARQKFSSLYISQFIIMYSLDGKKWQTYRGNSTGTLMVFFGNVDSSGIKHNIFNPPIIARYIRLHPTHYSIRSTLRMELMGCDLNSCSMPLGMESKAISDAQITASSYFTNMFATWSPSKARLHLQGRSNAWRPQVNNPKEWLQVDFQKTMKVTGVTTQGVKSLLTSMYVKEFLISSSQDGHQWTLFFQNGKVKVFQGNQDSFTPVVNSLDPPLLTRYLRIHPQSWVHQIALRMEVLGCEAQDLY

SEQ ID NO: 16 - protein, 1652 aa, synthetic construct
MQIELSTCFFLCLLRFCFSATRRYYLGAVELSWDYMQSDLGELPVDARFPPRVPKSFPFNTSVVYKKTLFVEFTDHLFNIAKPRPPWMGLLGPTIQAEVYDTVVITLKNMASHPVSLHAVGVSYWKASEGAEYDDQTSQREKEDDKVFPGGSHTYVWQVLKENGPMASDPLCLTYSYLSHVDLVKDLNSGLIGALLVCREGSLAKEKTQTLHKFILLFAVFDEGKSWHSETKNSLMQDRDAASARAWPKMHTVNGYVNRSLPGLIGCHRKSVYWHVIGMGTTPEVHSIFLEGHTFLVRNHRQASLEISPITFLTAQTLLMDLGQFLLFCHISSHQHDGMEAYVKVDSCPEEPQLRMKNNEEAEDYDDDLTDSEMDVVRFDDDNSPSFIQIRSVAKKHPKTWVHYIAAEEEDWDYAPLVLAPDDRSYKSQYLNNGPQRIGRKYKKVRFMAYTDETFKTREAIQHESGILGPLLYGEVGDTLLIIFKNQASRPYNIYPHGITDVRPLYSRRLPKGVKHLKDFPILPGEIFKYKWTVTVEDGPTKSDPRCLTRYYSSFVNMERDLASGLIGPLLICYKESVDQRGNQIMSDKRNVILFSVFDENRSWYLTENIQRFLPNPAGVQLEDPEFQASNIMHSINGYVFDSLQLSVCLHEVAYWYILSIGAQTDFLSVFFSGYTFKHKMVYEDTLTLFPFSGETVFMSMENPGLWILGCHNSDFRNRGMTALLKVSSCDKNTGDYYEDSYEDISAYLLSKNNAIEQRSFSQNSRHPSTRQKQFNATTIPENDIEKTDPWFAHRTPMPKIQNVSSSDLLMLLRQSPTPHGLSLSDLQEAKYETFSDDPSPGAIDSNNSLSEMTHFRPQLHHSGDMVFTPESGLQLRLNEKLGTTAATELKKLDFKVSSTSNNLISTIPSDNLAAGTDNTSSLGPPSMPVHYDSQLDTTLFGKKSSPLTESGGPLSLSEENNDSKLTREITRTTLQSDQEEIDYDDTISVEMKKEDFDIYDEDENQSPRSFQKKTRHYFIAAVERLWDYGMSSSPHVLRNRAQSGSVPQFKKVVFQEFTDGSFTQPLYRGELNEHLGLLGPYIRAEVEDNIMVTFRNQASRPYSFYSSLISYEEDQRQGAEPRKNFVKPNETKTYFWKVQHHMAPTKDEFDCKAWAYFSDVDLEKDVHSGLIGPLLVCHTNTLNPAHGRQVTVQEFALFFTIFDETKSWYFTENMERNCRAPCNIQMEDPTFKENYRFHAINGYIMDTLPGLVMAQDQRIRWYLLSMGSNENIHSIHFSGHVFTVRKKEEYKMALYNLYPGVFETVEMLPSKAGIWRVECLIGEHLHAGMSTLFLVYSNKCQTPLGMASGHIRDFQITASGQYGQWAPKLARLHYSGSINAWSTKEPFSWIKVDLLAPMIIHGIKTQGARQKFSSLYISQFIIMYSLDGKKWQTYRGNSTGTLMVFFGNVDSSGIKHNIFNPPIIARYIRLHPTHYSIRSTLRMELMGCDLNSCSMPLGMESKAISDAQITASSYFTNMFATWSPSKARLHLQGRSNAWRPQVNNPKEWLQVDFQKTMKVTGVTTQGVKSLLTSMYVKEFLISSSQDGHQWTLFFQNGKVKVFQGNQDSFTPVVNSLDPPLLTRYLRIHPQSWVHQIALRMEVLGCEAQDLY

SEQ ID NO: 17 - DNA, 4959 bp, synthetic construct
  source 1..4959: mol_type = other DNA
atgcagatcgagctgtctacctgcttcttcctgtgcctgctgcggttctgcttcagcgccaccagaagatattacctgggcgccgtggaactgagctgggactacatgcagtctgacctgggagagctgcccgtggacgctagatttcctccaagagtgcccaagagcttccccttcaacacctccgtggtgtacaagaaaaccctgttcgtggaattcaccgaccacctgttcaatatcgccaagcctcggcctccttggatgggactgctgggacctacaattcaggccgaggtgtacgacaccgtggtcatcaccctgaagaacatggccagccatcctgtgtctctgcacgccgtgggagtgtcttactggaaggcttctgagggcgccgagtacgacgatcagacaagccagagagagaaagaggacgacaaggttttccctggcggcagccacacctatgtctggcaggtcctgaaagaaaacggccctatggcctccgatcctctgtgcctgacatacagctacctgagccacgtggacctggtcaaggacctgaattctggcctgatcggagccctgctcgtgtgtagagaaggcagcctggccaaagagaaaacccagacactgcacaagttcatcctgctgttcgccgtgttcgacgagggcaagagctggcacagcgagacaaagaacagcctgatgcaggacagggatgccgcctctgctagagcttggcctaagatgcacaccgtgaacggctacgtgaacagaagcctgcctggactgatcggctgccacagaaagtccgtgtactggcacgtgatcggcatgggcacaacacctgaggtgcacagcatctttctggaaggacacaccttcctcgtgcggaaccatagacaggccagcctggaaatcagccctatcaccttcctgaccgctcagaccctgctgatggatctgggccagtttctgctgttctgccacatcagctcccaccagcacgatggcatggaagcctacgtgaaggtggacagctgccccgaagaaccccagctgcggatgaagaacaacgaggaagccgaggactacgacgacgacctgaccgactctgagatggacgtcgtcagattcgacgacgataacagccccagcttcatccagatcagaagcgtggccaagaagcaccccaagacctgggtgcactatatcgccgccgaggaagaggactgggattacgctcctctggtgctggcccctgacgacagaagctacaagagccagtacctgaacaacggccctcagcggatcggccggaagtataagaaagtgcggttcatggcctacaccgacgagacattcaagaccagagaggccatccagcacgagagcggaattctgggccctctgctgtatggcgaagtgggcgatacactgctgatcatcttcaagaaccaggccagcagaccctacaacatctaccctcacggcatcaccgatgtgcggcccctgtattctagaaggctgcccaagggcgtgaagcacctgaaggacttccctatcctgcctggcgagatcttcaagtacaagtggaccgtgaccgtggaagatggccccaccaagagcgaccctagatgtctgacacggtactacagcagcttcgtgaacatggaacgcgacctggccagcggcctgattggacctctgctgatctgctacaaagaaagcgtggaccagcggggcaaccagatcatgagcgacaagcggaacgtgatcctgtttagcgtgttcgatgagaaccggtcctggtatctgaccgagaacatccagcggtttctgcccaatcctgctggcgtgcagctggaagatcctgagttccaggcctccaacatcatgcactccatcaatggctatgtgttcgacagcctgcagctgagcgtgtgcctgcacgaagtggcctactggtacatcctgagcattggcgcccagaccgacttcctgtccgtgttctttagcggctacaccttcaagcacaagatggtgtacgaggataccctgacactgttcccattcagcggcgagacagtgttcatgagcatggaaaaccccggcctgtggatcctgggctgtcacaacagcgacttccggaacagaggcatgacagccctgctgaaggtgtccagctgcgacaagaacaccggcgactactacgaggacagctatgaggacatcagcgcctacctgctgagcaagaacaatgccatcgagagcagaagcttcagccagaatagcagacacccctccaccagacagaagcagttcaacgccacaacaatccccgagaacgacatcgagaaaaccgatccttggtttgcccacagaacccctatgcctaagatccagaacgtgtcctccagcgatctgctgatgctcctgagacagagccctacacctcacggactgagcctgtccgatctgcaagaggccaaatacgaaaccttcagcgacgacccttctcctggcgccatcgacagcaacaatagcctgagcgagatgacccacttcagaccacagctgcaccacagcggcgacatggtgtttacacctgagagcggcctccagctgagactgaatgagaagctgggaaccaccgccgccaccgagctgaagaaactggacttcaaggtgtcctctaccagcaacaacctgatcagcacaatcccctccgacaacctggctgccggcaccgacaacacatcttctctgggcccacctagcatgcccgtgcactacgatagccagctggataccacactgttcggcaagaagtctagccctctgacagagtctggcggccctctgtctctgagcgaggaaaacaacgacagcaagctgacccgcgagatcaccagaaccacactgcagagcgaccaagaggaaatcgattacgacgacaccatcagcgtcgagatgaagaaagaagatttcgacatctacgacgaggacgagaatcagagccccagaagctttcagaaaaagacccggcactacttcattgccgccgtcgagagactgtgggactacggcatgtctagcagccctcacgtgctgagaaatagagcccagagcggcagcgtgccccagttcaagaaagtggtgttccaagagttcaccgacggcagcttcacccagccactgtatagaggcgagctgaacgagcatctgggcctgctgggcccttatatcagagccgaagtggaagataacatcatggtcaccttccggaatcaggcctctcggccctacagcttctacagctccctgatctcctacgaagaggaccagagacagggcgctgagcccagaaagaacttcgtgaagcccaacgagactaagacctacttttggaaggtgcagcaccacatggcccctacaaaggacgagttcgactgcaaggcctgggcctacttttccgatgtggatctggaaaaggacgtgcacagcgggctcatcggaccactgcttgtgtgccacaccaacacactgaaccccgctcacggcagacaagtgacagtgcaagagttcgccctgttcttcaccatcttcgacgaaacaaagagctggtacttcaccgagaatatggaacggaactgtcgggccccttgcaacatccagatggaagatcccaccttcaaagagaactaccggttccacgccatcaacggctacatcatggacacactgcccggcctggttatggctcaggatcagagaatccggtggtatctgctgtccatgggctccaacgagaatatccacagcatccacttcagcggccacgtgttcaccgtgcggaaaaaagaagagtacaaaatggccctgtacaatctgtaccctggggtgttcgaaaccgtggaaatgctgccttccaaggccggcatttggagagtggaatgtctgattggagagcacctccacgccggaatgagcaccctgtttctggtgtactccaacaagtgtcagacccctctcggcatggcctctggacacatcagagacttccagatcaccgcctctggccagtacggacagtgggctcctaaactggctcggctgcactactccggcagcatcaatgcctggtccaccaaagagcccttcagctggatcaaggtggacctgctggctcccatgatcatccacggaatcaagacccagggcgcaagacagaagttcagcagcctgtacatcagccagttcatcatcatgtacagcctggacggaaagaagtggcagacctaccggggcaatagcaccggcacactcatggtgttcttcggcaacgtggactccagcggcattaagcacaacatcttcaaccctccaatcattgcccggtacatccggctgcaccccacacactacagcatccggtctaccctgagaatggaactgatgggctgcgacctgaacagctgcagcatgcccctcggaatggaaagcaaggccatcagcgacgcccagatcacagccagcagctacttcaccaacatgttcgccacttggagcccctccaaggctagactgcatctgcagggcagaagcaacgcttggaggccccaagtgaacaaccccaaagagtggctgcaggtcgactttcaaaagaccatgaaagtgaccggcgtgaccacacagggcgtcaagtctctgctgacctctatgtacgtgaaagagttcctgattagcagcagccaggacggccaccagtggaccctgtttttccagaacggcaaagtgaaagtgttccagggcaatcaggacagcttcacacccgtggtcaactccctggatcctccactgctgaccagatacctgcggattcaccctcagtcttgggtgcaccagatcgctctgcggatggaagtgctgggctgtgaagctcaggacctctactga

SEQ ID NO: 18 - DNA, 4959 bp, synthetic construct
  source 1..4959: mol_type = other DNA
atgcagatcgagctgtctacctgcttcttcctgtgcctgctgcggttctgcttcagcgccaccagaagatattacctgggcgccgtggaactgagctgggactacatgcagtctgacctgggagagctgcccgtggacgctagatttcctccaagagtgcccaagagcttccccttcaacacctccgtggtgtacaagaaaaccctgttcgtggaattcaccgaccacctgttcaatatcgccaagcctcggcctccttggatgggactgctgggacctacaattcaggccgaggtgtacgacaccgtggtcatcaccctgaagaacatggccagccatcctgtgtctctgcacgccgtgggagtgtcttactggaaggcttctgagggcgccgagtacgacgatcagacaagccagagagagaaagaggacgacaaggttttccctggcggcagccacacctatgtctggcaggtcctgaaagaaaacggccctatggcctccgatcctctgtgcctgacatacagctacctgagccacgtggacctggtcaaggacctgaattctggcctgatcggagccctgctcgtgtgtagagaaggcagcctggccaaagagaaaacccagacactgcacaagttcatcctgctgttcgccgtgttcgacgagggcaagagctggcacagcgagacaaagaacagcctgatgcaggacagggatgccgcctctgctagagcttggcctaagatgcacaccgtgaacggctacgtgaacagaagcctgcctggactgatcggctgccacagaaagtccgtgtactggcacgtgatcggcatgggcacaacacctgaggtgcacagcatctttctggaaggacacaccttcctcgtgcggaaccatagacaggccagcctggaaatcagccctatcaccttcctgaccgctcagaccctgctgatggatctgggccagtttctgctgttctgccacatcagctcccaccagcacgatggcatggaagcctacgtgaaggtggacagctgccccgaagaaccccagctgcggatgaagaacaacgaggaagccgaggactacgacgacgacctgaccgactctgagatggacgtcgtcagattcgacgacgataacagccccagcttcatccagatcagaagcgtggccaagaagcaccccaagacctgggtgcactatatcgccgccgaggaagaggactgggattacgctcctctggtgctggcccctgacgacagaagctacaagagccagtacctgaacaacggccctcagcggatcggccggaagtataagaaagtgcggttcatggcctacaccgacgagacattcaagaccagagaggccatccagcacgagagcggaattctgggccctctgctgtatggcgaagtgggcgatacactgctgatcatcttcaagaaccaggccagcagaccctacaacatctaccctcacggcatcaccgatgtgcggcccctgtattctagaaggctgcccaagggcgtgaagcacctgaaggacttccctatcctgcctggcgagatcttcaagtacaagtggaccgtgaccgtggaagatggccccaccaagagcgaccctagatgtctgacacggtactacagcagcttcgtgaacatggaacgcgacctggccagcggcctgattggacctctgctgatctgctacaaagaaagcgtggaccagcggggcaaccagatcatgagcgacaagcggaacgtgatcctgtttagcgtgttcgatgagaaccggtcctggtatctgaccgagaacatccagcggtttctgcccaatcctgctggcgtgcagctggaagatcctgagttccaggcctccaacatcatgcactccatcaatggctatgtgttcgacagcctgcagctgagcgtgtgcctgcacgaagtggcctactggtacatcctgagcattggcgcccagaccgacttcctgtccgtgttctttagcggctacaccttcaagcacaagatggtgtacgaggataccctgacactgttcccattcagcggcgagacagtgttcatgagcatggaaaaccccggcctgtggatcctgggctgtcacaacagcgacttccggaacagaggcatgacagccctgctgaaggtgtccagctgcgacaagaacaccggcgactactacgaggacagctatgaggacatcagcgcctacctgctgagcaagaacaatgccatcgagaacagaagcttcagccagaatagcagacacccctccaccagacagaagcagttcaacgccacaacaatccccgagaacgacatcgagaaaaccgatccttggtttgcccacagaacccctatgcctaagatccagaacgtgtcctccagcgatctgctgatgctcctgagacagagccctacacctcacggactgagcctgtccgatctgcaagaggccaaatacgaaaccttcagcgacgacccttctcctggcgccatcgacagcaacaatagcctgagcgagatgacccacttcagaccacagctgcaccacagcggcgacatggtgtttacacctgagagcggcctccagctgagactgaatgagaagctgggaaccaccgccgccaccgagctgaagaaactggacttcaaggtgtcctctaccagcaacaacctgatcagcacaatcccctccgacaacctggctgccggcaccgacaacacatcttctctgggcccacctagcatgcccgtgcactacgatagccagctggataccacactgttcggcaagaagtctagccctctgacagagtctggcggccctctgtctctgagcgaggaaaacaacgacagcaagctgacccgcgagatcaccagaaccacactgcagagcgaccaagaggaaatcgattacgacgacaccatcagcgtcgagatgaagaaagaagatttcgacatctacgacgaggacgagaatcagagccccagaagctttcagaaaaagacccggcactacttcattgccgccgtcgagagactgtgggactacggcatgtctagcagccctcacgtgctgagaaatagagcccagagcggcagcgtgccccagttcaagaaagtggtgttccaagagttcaccgacggcagcttcacccagccactgtatagaggcgagctgaacgagcatctgggcctgctgggcccttatatcagagccgaagtggaagataacatcatggtcaccttccggaatcaggcctctcggccctacagcttctacagctccctgatctcctacgaagaggaccagagacagggcgctgagcccagaaagaacttcgtgaagcccaacgagactaagacctacttttggaaggtgcagcaccacatggcccctacaaaggacgagttcgactgcaaggcctgggcctacttttccgatgtggatctggaaaaggacgtgcacagcgggctcatcggaccactgcttgtgtgccacaccaacacactgaaccccgctcacggcagacaagtgacagtgcaagagttcgccctgttcttcaccatcttcgacgaaacaaagagctggtacttcaccgagaatatggaacggaactgtcgggccccttgcaacatccagatggaagatcccaccttcaaagagaactaccggttccacgccatcaacggctacatcatggacacactgcccggcctggttatggctcaggatcagagaatccggtggtatctgctgtccatgggctccaacgagaatatccacagcatccacttcagcggccacgtgttcaccgtgcggaaaaaagaagagtacaaaatggccctgtacaatctgtaccctggggtgttcgaaaccgtggaaatgctgccttccaaggccggcatttggagagtggaatgtctgattggagagcacctccacgccggaatgagcaccctgtttctggtgtactccaacaagtgtcagacccctctcggcatggcctctggacacatcagagacttccagatcaccgcctctggccagtacggacagtgggctcctaaactggctcggctgcactactccggcagcatcaatgcctggtccaccaaagagcccttcagctggatcaaggtggacctgctggctcccatgatcatccacggaatcaagacccagggcgcaagacagaagttcagcagcctgtacatcagccagttcatcatcatgtacagcctggacggaaagaagtggcagacctaccggggcaatagcaccggcacactcatggtgttcttcggcaacgtggactccagcggcattaagcacaacatcttcaaccctccaatcattgcccggtacatccggctgcaccccacacactacagcatccggtctaccctgagaatggaactgatgggctgcgacctgaacagctgcagcatgcccctcggaatggaaagcaaggccatcagcgacgcccagatcacagccagcagctacttcaccaacatgttcgccacttggagcccctccaaggctagactgcatctgcagggcagaagcaacgcttggaggccccaagtgaacaaccccaaagagtggctgcaggtcgactttcaaaagaccatgaaagtgaccggcgtgaccacacagggcgtcaagtctctgctgacctctatgtacgtgaaagagttcctgattagcagcagccaggacggccaccagtggaccctgtttttccagaacggcaaagtgaaagtgttccagggcaatcaggacagcttcacacccgtggtcaactccctggatcctccactgctgaccagatacctgcggattcaccctcagtcttgggtgcaccagatcgctctgcggatggaagtgctgggctgtgaagctcaggacctctactga

SEQ ID NO: 19 - DNA, 4959 bp, synthetic construct
  source 1..4959: mol_type = other DNA
atgcagatcgagctgtctacctgcttcttcctgtgcctgctgcggttctgcttcagcgccaccagaagatattacctgggcgccgtggaactgagctgggactacatgcagtctgacctgggagagctgcccgtggacgctagatttcctccaagagtgcccaagagcttccccttcaacacctccgtggtgtacaagaaaaccctgttcgtggaattcaccgaccacctgttcaatatcgccaagcctcggcctccttggatgggactgctgggacctacaattcaggccgaggtgtacgacaccgtggtcatcaccctgaagaacatggccagccatcctgtgtctctgcacgccgtgggagtgtcttactggaaggcttctgagggcgccgagtacgacgatcagacaagccagagagagaaagaggacgacaaggttttccctggcggcagccacacctatgtctggcaggtcctgaaagaaaacggccctatggcctccgatcctctgtgcctgacatacagctacctgagccacgtggacctggtcaaggacctgaattctggcctgatcggagccctgctcgtgtgtagagaaggcagcctggccaaagagaaaacccagacactgcacaagttcatcctgctgttcgccgtgttcgacgagggcaagagctggcacagcgagacaaagaacagcctgatgcaggacagggatgccgcctctgctagagcttggcctaagatgcacaccgtgaacggctacgtgaacagaagcctgcctggactgatcggctgccacagaaagtccgtgtactggcacgtgatcggcatgggcacaacacctgaggtgcacagcatctttctggaaggacacaccttcctcgtgcggaaccatagacaggccagcctggaaatcagccctatcaccttcctgaccgctcagaccctgctgatggatctgggccagtttctgctgttctgccacatcagctcccaccagcacgatggcatggaagcctacgtgaaggtggacagctgccccgaagaaccccagctgcggatgaagaacaacgaggaagccgaggactacgacgacgacctgaccgactctgagatggacgtcgtcagattcgacgacgataacagccccagcttcatccagatcagaagcgtggccaagaagcaccccaagacctgggtgcactatatcgccgccgaggaagaggactgggattacgctcctctggtgctggcccctgacgacagaagctacaagagccagtacctgaacaacggccctcagcggatcggccggaagtataagaaagtgcggttcatggcctacaccgacgagacattcaagaccagagaggccatccagcacgagagcggaattctgggccctctgctgtatggcgaagtgggcgatacactgctgatcatcttcaagaaccaggccagcagaccctacaacatctaccctcacggcatcaccgatgtgcggcccctgtattctagaaggctgcccaagggcgtgaagcacctgaaggacttccctatcctgcctggcgagatcttcaagtacaagtggaccgtgaccgtggaagatggccccaccaagagcgaccctagatgtctgacacggtactacagcagcttcgtgaacatggaacgcgacctggccagcggcctgattggacctctgctgatctgctacaaagaaagcgtggaccagcggggcaaccagatcatgagcgacaagcggaacgtgatcctgtttagcgtgttcgatgagaaccggtcctggtatctgaccgagaacatccagcggtttctgcccaatcctgctggcgtgcagctggaagatcctgagttccaggcctccaacatcatgcactccatcaatggctatgtgttcgacagcctgcagctgagcgtgtgcctgcacgaagtggcctactggtacatcctgagcattggcgcccagaccgacttcctgtccgtgttctttagcggctacaccttcaagcacaagatggtgtacgaggataccctgacactgttcccattcagcggcgagacagtgttcatgagcatggaaaaccccggcctgtggatcctgggctgtcacaacagcgacttccggaacagaggcatgacagccctgctgaaggtgtccagctgcgacaagaacaccggcgactactacgaggacagctatgaggacatcagcgcctacctgctgagcaagaacaatgccatcgagcagagaagcttcagccagaatagcagacacccctccaccagacagaagcagttcaacgccacaacaatccccgagaacgacatcgagaaaaccgatccttggtttgcccacagaacccctatgcctaagatccagaacgtgtcctccagcgatctgctgatgctcctgagacagagccctacacctcacggactgagcctgtccgatctgcaagaggccaaatacgaaaccttcagcgacgacccttctcctggcgccatcgacagcaacaatagcctgagcgagatgacccacttcagaccacagctgcaccacagcggcgacatggtgtttacacctgagagcggcctccagctgagactgaatgagaagctgggaaccaccgccgccaccgagctgaagaaactggacttcaaggtgtcctctaccagcaacaacctgatcagcacaatcccctccgacaacctggctgccggcaccgacaacacatcttctctgggcccacctagcatgcccgtgcactacgatagccagctggataccacactgttcggcaagaagtctagccctctgacagagtctggcggccctctgtctctgagcgaggaaaacaacgacagcaagctgacccgcgagatcaccagaaccacactgcagagcgaccaagaggaaatcgattacgacgacaccatcagcgtcgagatgaagaaagaagatttcgacatctacgacgaggacgagaatcagagccccagaagctttcagaaaaagacccggcactacttcattgccgccgtcgagagactgtgggactacggcatgtctagcagccctcacgtgctgagaaatagagcccagagcggcagcgtgccccagttcaagaaagtggtgttccaagagttcaccgacggcagcttcacccagccactgtatagaggcgagctgaacgagcatctgggcctgctgggcccttatatcagagccgaagtggaagataacatcatggtcaccttccggaatcaggcctctcggccctacagcttctacagctccctgatctcctacgaagaggaccagagacagggcgctgagcccagaaagaacttcgtgaagcccaacgagactaagacctacttttggaaggtgcagcaccacatggcccctacaaaggacgagttcgactgcaaggcctgggcctacttttccgatgtggatctggaaaaggacgtgcacagcgggctcatcggaccactgcttgtgtgccacaccaacacactgaaccccgctcacggcagacaagtgacagtgcaagagttcgccctgttcttcaccatcttcgacgaaacaaagagctggtacttcaccgagaatatggaacggaactgtcgggccccttgcaacatccagatggaagatcccaccttcaaagagaactaccggttccacgccatcaacggctacatcatggacacactgcccggcctggttatggctcaggatcagagaatccggtggtatctgctgtccatgggctccaacgagaatatccacagcatccacttcagcggccacgtgttcaccgtgcggaaaaaagaagagtacaaaatggccctgtacaatctgtaccctggggtgttcgaaaccgtggaaatgctgccttccaaggccggcatttggagagtggaatgtctgattggagagcacctccacgccggaatgagcaccctgtttctggtgtactccaacaagtgtcagacccctctcggcatggcctctggacacatcagagacttccagatcaccgcctctggccagtacggacagtgggctcctaaactggctcggctgcactactccggcagcatcaatgcctggtccaccaaagagcccttcagctggatcaaggtggacctgctggctcccatgatcatccacggaatcaagacccagggcgcaagacagaagttcagcagcctgtacatcagccagttcatcatcatgtacagcctggacggaaagaagtggcagacctaccggggcaatagcaccggcacactcatggtgttcttcggcaacgtggactccagcggcattaagcacaacatcttcaaccctccaatcattgcccggtacatccggctgcaccccacacactacagcatccggtctaccctgagaatggaactgatgggctgcgacctgaacagctgcagcatgcccctcggaatggaaagcaaggccatcagcgacgcccagatcacagccagcagctacttcaccaacatgttcgccacttggagcccctccaaggctagactgcatctgcagggcagaagcaacgcttggaggccccaagtgaacaaccccaaagagtggctgcaggtcgactttcaaaagaccatgaaagtgaccggcgtgaccacacagggcgtcaagtctctgctgacctctatgtacgtgaaagagttcctgattagcagcagccaggacggccaccagtggaccctgtttttccagaacggcaaagtgaaagtgttccagggcaatcaggacagcttcacacccgtggtcaactccctggatcctccactgctgaccagatacctgcggattcaccctcagtcttgggtgcaccagatcgctctgcggatggaagtgctgggctgtgaagctcaggacctctactga

SEQ ID NO: 20 - DNA, 20 bp, synthetic construct
  source 1..20: mol_type = other DNA
gtgcggcccctgtattctag

SEQ ID NO: 21 - DNA, 21 bp, synthetic construct
  source 1..21: mol_type = other DNA
cttctgctctcgatggcattg

SEQ ID NO: 22 - DNA, 22 bp, synthetic construct
  source 1..22: mol_type = other DNA
catcgagagcagaagcttcagc

SEQ ID NO: 23 - DNA, 22 bp, synthetic construct
  source 1..22: mol_type = other DNA
gttgattgttccagacgcgttc

SEQ ID NO: 24 - DNA, 21 bp, synthetic construct
  source 1..21: mol_type = other DNA
cttctgttctcgatggcattg

SEQ ID NO: 25 - DNA, 22 bp, synthetic construct
  source 1..22: mol_type = other DNA
catcgagaacagaagcttcagc

SEQ ID NO: 26 - DNA, 21 bp, synthetic construct
  source 1..21: mol_type = other DNA
cttctctgctcgatggcattg

SEQ ID NO: 27 - DNA, 22 bp, synthetic construct
  source 1..22: mol_type = other DNA
catcgagcagagaagcttcagc

SEQ ID NO: 28 - protein, 2813 aa, Homo sapiens
MIPARFAGVLLALALILPGTLCAEGTRGRSSTARCSLFGSDFVNTFDGSMYSFAGYCSYLLAGGCQKRSFSIIGDFQNGKRVSLSVYLGEFFDIHLFVNGTVTQGDQRVSMPYASKGLYLETEAGYYKLSGEAYGFVARIDGSGNFQVLLSDRYFNKTCGLCGNFNIFAEDDFMTQEGTLTSDPYDFANSWALSSGEQWCERASPPSSSCNISSGEMQKGLWEQCQLLKSTSVFARCHPLVDPEPFVALCEKTLCECAGGLECACPALLEYARTCAQEGMVLYGWTDHSACSPVCPAGMEYRQCVSPCARTCQSLHINEMCQERCVDGCSCPEGQLLDEGLCVESTECPCVHSGKRYPPGTSLSRDCNTCICRNSQWICSNEECPGECLVTGQSHFKSFDNRYFTFSGICQYLLARDCQDHSFSIVIETVQCADDRDAVCTRSVTVRLPGLHNSLVKLKHGAGVAMDGQDVQLPLLKGDLRIQHTVTASVRLSYGEDLQMDWDGRGRLLVKLSPVYAGKTCGLCGNYNGNQGDDFLTPSGLAEPRVEDFGNAWKLHGDCQDLQKQHSDPCALNPRMTRFSEEACAVLTSPTFEACHRAVSPLPYLRNCRYDVCSCSDGRECLCGALASYAAACAGRGVRVAWREPGRCELNCPKGQVYLQCGTPCNLTCRSLSYPDEECNEACLEGCFCPPGLYMDERGDCVPKAQCPCYYDGEIFQPEDIFSDHHTMCYCEDGFMHCTMSGVPGSLLPDAVLSSPLSHRSKRSLSCRPPMVKLVCPADNLRAEGLECTKTCQNYDLECMSMGCVSGCLCPPGMVRHENRCVALERCPCFHQGKEYAPGETVKIGCNTCVCQDRKWNCTDHVCDATCSTIGMAHYLTFDGLKYLFPGECQYVLVQDYCGSNPGTFRILVGNKGCSHPSVKCKKRVTILVEGGEIELFDGEVNVKRPMKDETHFEVVESGRYIILLLGKALSVVWDRHLSISVVLKQTYQEKVCGLCGNFDGIQNNDLTSSNLQVEEDPVDFGNSWKVSSQCADTRKVPLDSSPATCHNNIMKQTMVDSSCRILTSDVFQDCNKLVDPEPYLDVCIYDTCSCESIGDCACFCDTIAAYAHVCAQHGKVVTWRTATLCPQSCEERNLRENGYECEWRYNSCAPACQVTCQHPEPLACPVQCVEGCHAHCPPGKILDELLQTCVDPEDCPVCEVAGRRFASGKKVTLNPSDPEHCQICHCDVVNLTCEACQEPGGLVVPPTDAPVSPTTLYVEDISEPPLHDFYCSRLLDLVFLLDGSSRLSEAEFEVLKAFVVDMMERLRISQKWVRVAVVEYHDGSHAYIGLKDRKRPSELRRIASQVKYAGSQVASTSEVLKYTLFQIFSKIDRPEASRITLLLMASQEPQRMSRNFVRYVQGLKKKKVIVIPVGIGPHANLKQIRLIEKQAPENKAFVLSSVDELEQQRDEIVSYLCDLAPEAPPPTLPPDMAQVTVGPGLLGVSTLGPKRNSMVLDVAFVLEGSDKIGEADFNRSKEFMEEVIQRMDVGQDSIHVTVLQYSYMVTVEYPFSEAQSKGDILQRVREIRYQGGNRTNTGLALRYLSDHSFLVSQGDREQAPNLVYMVTGNPASDEIKRLPGDIQVVPIGVGPNANVQELERIGWPNAPILIQDFETLPREAPDLVLQRCCSGEGLQIPTLSPAPDCSQPLDVILLLDGSSSFPASYFDEMKSFAKAFISKANIGPRLTQVSVLQYGSITTIDVPWNVVPEKAHLLSLVDVMQREGGPSQIGDALGFAVRYLTSEMHGARPGASKAVVILVTDVSVDSVDAAADAARSNRVTVFPIGIGDRYDAAQLRILAGPAGDSNVVKLQRIEDLPTMVTLGNSFLHKLCSGFVRICMDEDGNEKRPGDVWTLPDQCHTVTCQPDGQTLLKSHRVNCDRGLRPSCPNSQSPVKVEETCGCRWTCPCVCTGSSTRHIVTFDGQNFKLTGSCSYVLFQNKEQDLEVILHNGACSPGARQGCMKSIEVKHSALSVELHSDMEVTVNGRLVSVPYVGGNMEVNVYGAIMHEVRFNHLGHIFTFTPQNNEFQLQLSPKTFASKTYGLCGICDENGANDFMLRDGTVTTDWKTLVQEWTVQRPGQTCQPILEEQCLVPDSSHCQVLLLPLFAECHKVLAPATFYAICQQDSCHQEQVCEVIASYAHLCRTNGVCVDWRTPDFCAMSCPPSLVYNHCEHGCPRHCDGNVSSCGDHPSEGCFCPPDKVMLEGSCVPEEACTQCIGEDGVQHQFLEAWVPDHQPCQICTCLSGRKVNCTTQPCPTAKAPTCGLCEVARLRQNADQCCPEYECVCDPVSCDLPPVPHCERGLQPTLTNPGECRPNFTCACRKEECKRVSPPSCPPHRLPTLRKTQCCDEYECACNCVNSTVSCPLGYLASTATNDCGCTTTTCLPDKVCVHRSTIYPVGQFWEEGCDVCTCTDMEDAVMGLRVAQCSQKPCEDSCRSGFTYVLHEGECCGRCLPSACEVVTGSPRGDSQSSWKSVGSQWASPENPCLINECVRVKEEVFIQQRNVSCPQLEVPVCPSGFQLSCKTSACCPSCRCERMEACMLNGTVIGPGKTVMIDVCTTCRCMVQVGVISGFKLECRKTTCNPCPLGYKEENNTGECCGRCLPTACTIQLRGGQIMTLKRDETLQDGCDTHFCKVNERGEYFWEKRVTGCPPFDEHKCLAEGGKIMKIPGTCCDTCEEPECNDITARLQYVKVGSCKSEVEVDIHYCQGKCASKAMYSIDINDVQDQCSCCSPTRTEPMQVALHCTNGSVVYHEVLNAMECKCSPRKCSK

SEQ ID NO: 29 - protein, 1421 aa, synthetic construct
MIPARFAGVLLALALILPGTLCAEGTRGRSSTARCSLFGSDFVNTFDGSMYSFAGYCSYLLAGGCQKRSFSIIGDFQNGKRVSLSVYLGEFFDIHLFVNGTVTQGDQRVSMPYASKGLYLETEAGYYKLSGEAYGFVARIDGSGNFQVLLSDRYFNKTCGLCGNFNIFAEDDFMTQEGTLTSDPYDFANSWALSSGEQWCERASPPSSSCNISSGEMQKGLWEQCQLLKSTSVFARCHPLVDPEPFVALCEKTLCECAGGLECACPALLEYARTCAQEGMVLYGWTDHSACSPVCPAGMEYRQCVSPCARTCQSLHINEMCQERCVDGCSCPEGQLLDEGLCVESTECPCVHSGKRYPPGTSLSRDCNTCICRNSQWICSNEECPGECLVTGQSHFKSFDNRYFTFSGICQYLLARDCQDHSFSIVIETVQCADDRDAVCTRSVTVRLPGLHNSLVKLKHGAGVAMDGQDVQLPLLKGDLRIQHTVTASVRLSYGEDLQMDWDGRGRLLVKLSPVYAGKTCGLCGNYNGNQGDDFLTPSGLAEPRVEDFGNAWKLHGDCQDLQKQHSDPCALNPRMTRFSEEACAVLTSPTFEACHRAVSPLPYLRNCRYDVCSCSDGRECLCGALASYAAACAGRGVRVAWREPGRCELNCPKGQVYLQCGTPCNLTCRSLSYPDEECNEACLEGCFCPPGLYMDERGDCVPKAQCPCYYDGEIFQPEDIFSDHHTMCYCEDGFMHCTMSGVPGSLLPDAVLSSPLSHRSKRSLSCRPPMVKLVCPADNLRAEGLECTKTCQNYDLECMSMGCVSGCLCPPGMVRHENRCVALERCPCFHQGKEYAPGETVKIGCNTCVCRDRKWNCTDHVCDATCSTIGMAHYLTFDGLKYLFPGECQYVLVQDYCGSNPGTFRILVGNKGCSHPSVKCKKRVTILVEGGEIELFDGEVNVKRPMKDETHFEVVESGRYIILLLGKALSVVWDRHLSISVVLKQTYQEKVCGLCGNFDGIQNNDLTSSNLQVEEDPVDFGNSWKVSSQCADTRKVPLDSSPATCHNNIMKQTMVDSSCRILTSDVFQDCNKLVDPEPYLDVCIYDTCSCESIGDCACFCDTIAAYAHVCAQHGKVVTWRTATLCPQSCEERNLRENGYECEWRYNSCAPACQVTCQHPEPLACPVQCVEGCHAHCPPGKILDELLQTCVDPEDCPVCEVAGRRFASGKKVTLNPSDPEHCQICHCDVVNLTCEACQEPGGLVVPPTDAPVSPTTLYVEDISEPPLHDFRDETLQDGCDTHFCKVNERGEYFWEKRVTGCPPFDEHKCLAEGGKIMKIPGTCCDTCEEPECNDITARLQYVKVGSCKSEVEVDIHYCQGKCASKAMYSIDINDVQDQCSCCSPTRTEPMQVALHCTNGSVVYHEVLNAMECKCSPRKCSK

SEQ ID NO: 30 - protein, 1268 aa, synthetic construct
MIPARFAGVLLALALILPGTLCAEGTRGRSSTARCSLFGSDFVNTFDGSMYSFAGYCSYLLAGGCQKRSFSIIGDFQNGKRVSLSVYLGEFFDIHLFVNGTVTQGDQRVSMPYASKGLYLETEAGYYKLSGEAYGFVARIDGSGNFQVLLSDRYFNKTCGLCGNFNIFAEDDFMTQEGTLTSDPYDFANSWALSSGEQWCERASPPSSSCNISSGEMQKGLWEQCQLLKSTSVFARCHPLVDPEPFVALCEKTLCECAGGLECACPALLEYARTCAQEGMVLYGWTDHSACSPVCPAGMEYRQCVSPCARTCQSLHINEMCQERCVDGCSCPEGQLLDEGLCVESTECPCVHSGKRYPPGTSLSRDCNTCICRNSQWICSNEECPGECLVTGQSHFKSFDNRYFTFSGICQYLLARDCQDHSFSIVIETVQCADDRDAVCTRSVTVRLPGLHNSLVKLKHGAGVAMDGQDIQLPLLKGDLRIQHTVTASVRLSYGEDLQMDWDGRGRLLVKLSPVYAGKTCGLCGNYNGNQGDDFLTPSGLAEPRVEDFGNAWKLHGDCQDLQKQHSDPCALNPRMTRFSEEACAVLTSPTFEACHRAVSPLPYLRNCRYDVCSCSDGRECLCGALASYAAACAGRGVRVAWREPGRCELNCPKGQVYLQCGTPCNLTCRSLSYPDEECNEACLEGCFCPPGLYMDERGDCVPKAQCPCYYDGEIFQPEDIFSDHHTMCYCEDGFMHCTMSGVPGSLLPDAVLSSPLSHRSKRSLSCRPPMVKLVCPADNLRAEGLECTKTCQNYDLECMSMGCVSGCLCPPGMVRHENRCVALERCPCFHQGKEYAPGETVKIGCNTCVCRDRKWNCTDHVCDATCSTIGMAHYLTFDGLKYLFPGECQYVLVQDYCGSNPGTFRILVGNKGCSHPSVKCKKRVTILVEGGEIELFDGEVNVKRPMKDETHFEVVESGRYIILLLGKALSVVWDRHLSISVVLKQTYQEKVCGLCGNFDGIQNNDLTSSNLQVEEDPVDFGNSWKVSSQCADTRKVPLDSSPATCHNNIMKQTMVDSSCRILTSDVFQDCNKLVDPEPYLDVCIYDTCSCESIGDCACFCDTIAAYAHVCAQHGKVVTWRTATLCPQSCEERNLRENGYECEWRYNSCAPACQVTCQHPEPLACPVQCVEGCHAHCPPGKILDELLQTCVDPEDCPVCEVAGRRFASGKKVTLNPSDPEHCQICHCDVVNLTCEACQEPGGLVVPPTDAPVSPTTLYVEDISEPPLH

SEQ ID NO: 31 - protein, 527 aa, synthetic construct
MIPARFAGVLLALALILPGTLCSLSCRPPMVKLVCPADNLRAEGLECTKTCQNYDLECMSMGCVSGCLCPPGMVRHENRCVALERCPCFHQGKEYAPGETVKIGCNTCVCRDRKWNCTDHVCDATCSTIGMAHYLTFDGLKYLFPGECQYVLVQDYCGSNPGTFRILVGNKGCSHPSVKCKKRVTILVEGGEIELFDGEVNVKRPMKDETHFEVVESGRYIILLLGKALSVVWDRHLSISVVLKQTYQEKVCGLCGNFDGIQNNDLTSSNLQVEEDPVDFGNSWKVSSQCADTRKVPLDSSPATCHNNIMKQTMVDSSCRILTSDVFQDCNKLVDPEPYLDVCIYDTCSCESIGDCACFCDTIAAYAHVCAQHGKVVTWRTATLCPQSCEERNLRENGYECEWRYNSCAPACQVTCQHPEPLACPVQCVEGCHAHCPPGKILDELLQTCVDPEDCPVCEVAGRRFASGKKVTLNPSDPEHCQICHCDVVNLTCEACQEPGGLVVPPTDAPVSPTTLYVEDISEPPLH

SEQ ID NO: 32 - DNA, 4266 bp, synthetic construct
  source 1..4266: mol_type = other DNA
atgattcctgccagatttgccggggtgctgcttgctctggccctcattttgccagggaccctttgtgcagaaggaactcgcggcaggtcatccacggcccgatgcagccttttcggaagtgacttcgtcaacacctttgatgggagcatgtacagctttgcgggatactgcagttacctcctggcagggggctgccagaaacgctccttctcgattattggggacttccagaatggcaagagagtgagcctctccgtgtatcttggggaattttttgacatccatttgtttgtcaatggtaccgtgacacagggggaccaaagagtctccatgccctatgcctccaaagggctgtatctagaaactgaggctgggtactacaagctgtccggtgaggcctatggctttgtggccaggatcgatggcagcggcaactttcaagtcctgctgtcagacagatacttcaacaagacctgcgggctgtgtggcaactttaacatctttgctgaagatgactttatgacccaagaagggaccttgacctcggacccttatgactttgccaactcatgggctctgagcagtggagaacagtggtgtgaacgggcatctcctcccagcagctcatgcaacatctcctctggggaaatgcagaagggcctgtgggagcagtgccagcttctgaagagcacctcggtgtttgcccgctgccaccctctggtggaccccgagccttttgtggccctgtgtgagaagactttgtgtgagtgtgctggggggctggagtgcgcctgccctgccctcctggagtacgcccggacctgtgcccaggagggaatggtgctgtacggctggaccgaccacagcgcgtgcagcccagtgtgccctgctggtatggagtataggcagtgtgtgtccccttgcgccaggacctgccagagcctgcacatcaatgaaatgtgtcaggagcgatgcgtggatggctgcagctgccctgagggacagctcctggatgaaggcctctgcgtggagagcaccgagtgtccctgcgtgcattccggaaagcgctaccctcccggcacctccctctctcgagactgcaacacctgcatttgccgaaacagccagtggatctgcagcaatgaagaatgtccaggggagtgccttgtcacaggtcaatcacacttcaagagctttgacaacagatacttcaccttcagtgggatctgccagtacctgctggcccgggattgccaggaccactccttctccattgtcattgagactgtccagtgtgctgatgaccgcgacgctgtgtgcacccgctccgtcaccgtccggctgcctggcctgcacaacagccttgtgaaactgaagcatggggcaggagttgccatggatggccaggacgtccagctccccctcctgaaaggtgacctccgcatccagcatacagtgacggcctccgtgcgcctcagctacggggaggacctgcagatggactgggatggccgcgggaggctgctggtgaagctgtcccccgtctatgccgggaagacctgcggcctgtgtgggaattacaatggcaaccagggcgacgacttccttaccccctctgggctggcggagccccgggtggaggacttcgggaacgcctggaagctgcacggggactgccaggacctgcagaagcagcacagcgatccctgcgccctcaacccgcgcatgaccaggttctccgaggaggcgtgcgcggtcctgacgtcccccacattcgaggcctgccatcgtgccgtcagcccgctgccctacctgcggaactgccgctacgacgtgtgctcctgctcggacggccgcgagtgcctgtgcggcgccctggccagctatgccgcggcctgcgcggggagaggcgtgcgcgtcgcgtggcgcgagccaggccgctgtgagctgaactgcccgaaaggccaggtgtacctgcagtgcgggaccccctgcaacctgacctgccgctctctctcttacccggatgaggaatgcaatgaggcctgcctggagggctgcttctgccccccagggctctacatggatgagaggggggactgcgtgcccaaggcccagtgcccctgttactatgacggtgagatcttccagccagaagacatcttctcagaccatcacaccatgtgctactgtgaggatggcttcatgcactgtaccatgagtggagtccccggaagcttgctgcctgacgctgtcctcagcagtcccctgtctcatcgcagcaaaaggagcctatcctgtcggccccccatggtcaagctggtgtgtcccgctgacaacctgcgggctgaagggctcgagtgtaccaaaacgtgccagaactatgacctggagtgcatgagcatgggctgtgtctctggctgcctctgccccccgggcatggtccggcatgagaacagatgtgtggccctggaaaggtgtccctgcttccatcagggcaaggagtatgcccctggagaaacagtgaagattggctgcaacacttgtgtctgtcgggaccggaagtggaactgcacagaccatgtgtgtgatgccacgtgctccacgatcggcatggcccactacctcaccttcgacgggctcaaatacctgttccccggggagtgccagtacgttctggtgcaggattactgcggcagtaaccctgggacctttcggatcctagtggggaataagggatgcagccacccctcagtgaaatgcaagaaacgggtcaccatcctggtggagggaggagagattgagctgtttgacggggaggtgaatgtgaagaggcccatgaaggatgagactcactttgaggtggtggagtctggccggtacatcattctgctgctgggcaaagccctctccgtggtctgggaccgccacctgagcatctccgtggtcctgaagcagacataccaggagaaagtgtgtggcctgtgtgggaattttgatggcatccagaacaatgacctcaccagcagcaacctccaagtggaggaagaccctgtggactttgggaactcctggaaagtgagctcgcagtgtgctgacaccagaaaagtgcctctggactcatcccctgccacctgccataacaacatcatgaagcagacgatggtggattcctcctgtagaatccttaccagtgacgtcttccaggactgcaacaagctggtggaccccgagccatatctggatgtctgcatttacgacacctgctcctgtgagtccattggggactgcgcctgcttctgcgacaccattgctgcctatgcccacgtgtgtgcccagcatggcaaggtggtgacctggaggacggccacattgtgcccccagagctgcgaggagaggaatctccgggagaacgggtatgagtgtgagtggcgctataacagctgtgcacctgcctgtcaagtcacgtgtcagcaccctgagccactggcctgccctgtgcagtgtgtggagggctgccatgcccactgccctccagggaaaatcctggatgagcttttgcagacctgcgttgaccctgaagactgtccagtgtgtgaggtggctggccggcgttttgcctcaggaaagaaagtcaccttgaatcccagtgaccctgagcactgccagatttgccactgtgatgttgtcaacctcacctgtgaagcctgccaggagccgggaggcctggtggtgcctcccacagatgccccggtgagccccaccactctgtatgtggaggacatctcggaaccgccgttgcacgatttccgtgatgagacgctccaggatggctgtgatactcacttctgcaaggtcaatgagagaggagagtacttctgggagaagagggtcacaggctgcccaccctttgatgaacacaagtgtctggctgagggaggtaaaattatgaaaattccaggcacctgctgtgacacatgtgaggagcctgagtgcaacgacatcactgccaggctgcagtatgtcaaggtgggaagctgtaagtctgaagtagaggtggatatccactactgccagggcaaatgtgccagcaaagccatgtactccattgacatcaacgatgtgcaggaccagtgctcctgctgctctccgacacggacggagcccatgcaggtggccctgcactgcaccaatggctctgttgtgtaccatgaggttctcaatgccatggagtgcaaatgctcccccaggaagtgcagcaagtga

SEQ ID NO: 33 - DNA, 3807 bp, synthetic construct
  source 1..3807: mol_type = other DNA
atgattccagccagatttgctggcgtgctgctggccctggctctgattcttcctggaacactgtgtgccgagggcaccagaggcagatctagcacagccagatgcagcctgttcggcagcgacttcgtgaacaccttcgacggcagcatgtacagcttcgccggctactgtagctacctgttggctggcggctgccagaagagaagcttcagcatcatcggcgacttccagaacggcaagagggtgtccctgtctgtgtacctgggcgagttcttcgacatccacctgttcgtgaacggcaccgtgacacagggcgaccagcgagtgtctatgccttacgcctctaagggcctgtacctggaaacagaggccggctattacaagctgagcggcgaggcctatggcttcgtggccagaatcgatggcagcggcaatttccaggtgctgctgagcgaccggtacttcaacaagacctgtggcctgtgcggcaacttcaacatcttcgccgaggacgacttcatgacccaagagggcaccctgaccagcgatccctacgactttgccaatagctgggccctgtctagcggagagcagtggtgtgaaagagcctctccacctagcagcagctgcaacatcagcagcggcgagatgcagaaaggcctgtgggaacagtgccagctgctgaagtctaccagcgtgttcgccagatgtcaccctctggtggaccctgagccttttgtggccctgtgtgaaaagaccctgtgcgagtgtgctggcggcctggaatgtgcttgtcctgctctgctggaatacgcccggacatgtgcccaagaaggcatggttctgtacggctggaccgaccactctgcctgctctccagtgtgtcctgccggcatggaatatcggcagtgcgtgtcaccttgcgccagaacctgtcagagcctgcacatcaacgagatgtgccaagaaagatgcgtggacggctgctcctgtcctgaaggacagctgctggatgagggcctgtgtgtggaaagcaccgagtgtccttgtgtgcacagcggcaagagataccctcctggcacaagcctgagccgggactgcaatacctgcatctgcagaaacagccagtggatctgcagcaacgaggaatgccctggcgagtgcctggttacaggccagagccacttcaagagcttcgacaacagatacttcaccttcagcggcatctgccagtacctgctggccagagattgccaggaccacagcttctccatcgtgatcgagacagtgcagtgcgccgacgacagagatgccgtgtgtaccagatctgtgaccgtgcgactgcccggcctgcacaattctctggtcaagctgaaacacggcgctggcgtggcaatggacggccaggatattcaactgcccctgctgaagggcgacctgagaattcagcataccgtgacagccagcgtgcggctgtcttatggcgaggacctgcagatggactgggatggaagaggcagactgctcgtgaagctgagccctgtgtacgccggcaagacatgcggactgtgtggcaattacaacggcaaccagggcgacgactttctgacaccttctggactggccgagcctagagtggaagatttcggcaacgcctggaagctgcacggcgactgtcaggatctgcaaaagcagcacagcgacccctgcgctctgaaccccagaatgaccagattcagcgaagaggcctgcgccgtgctgacaagccctacatttgaggcctgccacagagccgtgtcacccctgccttacctgcggaactgcagatacgacgtgtgcagctgtagcgacggccgggaatgtctttgtggcgccctggcttcttatgccgccgcttgtgccggaagaggcgttagagttgcttggagagaacccggcagatgcgagctgaactgccctaaaggacaggtgtacctgcagtgcggcaccccttgcaacctgacctgtagatccctgagctaccccgacgaagagtgcaacgaggcctgtctggaaggctgcttctgccctcctggactgtacatggatgagaggggcgattgcgtgcccaaggctcagtgcccttgttactacgacggcgagatcttccagcctgaggacatcttcagcgaccaccacaccatgtgctactgcgaggatggcttcatgcactgcaccatgagcggcgtgccaggatctctgctgcctgatgctgttctgagcagccctctgagccacagaagcaagagaagcctgagctgcagacctcctatggtcaagctcgtgtgccctgccgacaacctgagagccgaaggcctggaatgcaccaagacctgccagaactacgacctcgagtgcatgagcatgggctgcgtgtccggatgtctgtgtcctcctggaatggtccgacacgagaacagatgcgtggccctggaacggtgcccttgcttccaccaaggcaaagagtatgcccctggcgagacagtgaagatcggctgcaatacctgcgtgtgccgggacagaaagtggaactgcaccgatcacgtgtgcgacgccacctgtagcacaatcggcatggcccactacctgaccttcgacggcctgaagtacctgtttcctggcgagtgccagtacgtgctggtgcaggattactgcggcagcaaccctggcaccttcagaatcctcgtgggcaacaagggctgctctcaccctagcgtgaagtgcaagaagcgggtcaccatcctggtggaaggcggagagatcgagctgttcgacggcgaagtgaacgtgaagcggcccatgaaggacgagacacacttcgaggtggtggaaagcggccggtacatcatcctgctgctgggcaaagccctgagcgtcgtgtgggatagacacctgagcatcagcgtggtgctgaagcagacctaccaagagaaagtgtgcggcctgtgcggcaacttcgatggcatccagaacaacgatctgaccagcagcaacctccaggtggaagaggaccctgtggacttcggcaacagctggaaggtgtccagccagtgcgccgacacaagaaaggtgccactggatagcagccccgccacatgccacaacaacatcatgaagcaaaccatggtggacagcagctgccggatcctgacctccgatgtgttccaggactgcaacaagctggtggaccccgagccttacctggacgtgtgcatctacgatacctgcagctgcgagagcatcggcgattgcgcctgcttctgcgatacaatcgccgcctacgctcatgtgtgcgcccagcacggaaaggtggtcacttggagaaccgccacactgtgtccacagagctgcgaggaacggaatctgcgcgagaatggctacgagtgcgagtggcggtacaatagctgtgcccctgcctgtcaagtgacctgtcagcaccctgagcctctggcttgtcctgtgcagtgtgtggaaggctgccacgctcattgtccacctggcaagatcctggacgagctgctgcagacatgtgtggatcccgaggattgccctgtgtgcgaagtggccggaagaagatttgccagcggcaagaaagtgaccctgaatcctagcgaccctgagcactgccagatctgccactgcgacgtggtcaatctgacatgcgaggcctgccaagaacctggcggactggttgtgcctcctacagatgctcctgtgtctcccaccacactgtacgtggaagatatcagcgagcctcctctgcactga

SEQ ID NO: 34 - DNA, 1584 bp, synthetic construct
  source 1..1584: mol_type = other DNA
atgatccctgccagatttgctggcgtgctgctggccctggctctgattcttcctggcacactgtgcagcctgagctgcagacctcctatggtcaagctcgtgtgccctgccgacaacctgagagccgaaggcctggaatgcaccaagacctgccagaactacgacctcgagtgcatgagcatgggctgcgtgtccggatgtctgtgtcctcctggaatggtccgacacgagaacagatgcgtggccctggaacggtgcccttgcttccaccaaggcaaagagtatgcccctggcgagacagtgaagatcggctgcaatacctgcgtgtgccgggacagaaagtggaactgcaccgatcacgtgtgcgacgccacctgtagcacaatcggcatggcccactacctgaccttcgacggcctgaagtacctgtttcctggcgagtgccagtacgtgctggtgcaggattactgcggcagcaaccctggcaccttcagaatcctcgtgggcaacaagggctgctctcaccctagcgtgaagtgcaagaagcgggtcaccatcctggtggaaggcggagagatcgagctgttcgacggcgaagtgaacgtgaagcggcccatgaaggacgagacacacttcgaggtggtggaaagcggccggtacatcatcctgctgctgggcaaagccctgagcgtcgtgtgggatagacacctgagcatcagcgtggtgctgaagcagacctaccaagagaaagtgtgcggcctgtgcggcaacttcgatggcatccagaacaacgatctgaccagcagcaacctccaggtggaagaggaccctgtggacttcggcaacagctggaaggtgtccagccagtgcgccgacacaagaaaggtgccactggatagcagccccgccacatgccacaacaacatcatgaagcaaaccatggtggacagcagctgccggatcctgacctccgatgtgttccaggactgcaacaagctggtggaccccgagccttacctggacgtgtgcatctacgatacctgcagctgcgagagcatcggcgattgcgcctgcttctgcgatacaatcgccgcctacgctcatgtgtgcgcccagcacggaaaggtggtcacttggagaaccgccacactgtgtccacagagctgcgaggaacggaatctgcgcgagaatggctacgagtgcgagtggcggtacaatagctgtgcccctgcctgtcaagtgacctgtcagcaccctgagcctctggcttgtcctgtgcagtgtgtggaaggctgccacgctcattgtccacctggcaagatcctggacgagctgctgcagacatgtgtggatcccgaggattgccctgtgtgcgaagtggccggaagaagatttgccagcggcaagaaagtgaccctgaatcctagcgaccctgagcactgccagatctgccactgcgacgtggtcaatctgacatgcgaggcctgccaagaacctggcggactggttgtgcctcctacagatgctcctgtgtctcccaccacactgtacgtggaagatatcagcgagcctcctctgcactga

SEQ ID NO: 35 - DNA, 8442 bp, Homo sapiens
  source 1..8442: mol_type = genomic DNA
atgattcctgccagatttgccggggtgctgcttgctctggccctcattttgccagggaccctttgtgcagaaggaactcgcggcaggtcatccacggcccgatgcagccttttcggaagtgacttcgtcaacacctttgatgggagcatgtacagctttgcgggatactgcagttacctcctggcagggggctgccagaaacgctccttctcgattattggggacttccagaatggcaagagagtgagcctctccgtgtatcttggggaattttttgacatccatttgtttgtcaatggtaccgtgacacagggggaccaaagagtctccatgccctatgcctccaaagggctgtatctagaaactgaggctgggtactacaagctgtccggtgaggcctatggctttgtggccaggatcgatggcagcggcaactttcaagtcctgctgtcagacagatacttcaacaagacctgcgggctgtgtggcaactttaacatctttgctgaagatgactttatgacccaagaagggaccttgacctcggacccttatgactttgccaactcatgggctctgagcagtggagaacagtggtgtgaacgggcatctcctcccagcagctcatgcaacatctcctctggggaaatgcagaagggcctgtgggagcagtgccagcttctgaagagcacctcggtgtttgcccgctgccaccctctggtggaccccgagccttttgtggccctgtgtgagaagactttgtgtgagtgtgctggggggctggagtgcgcctgccctgccctcctggagtacgcccggacctgtgcccaggagggaatggtgctgtacggctggaccgaccacagcgcgtgcagcccagtgtgccctgctggtatggagtataggcagtgtgtgtccccttgcgccaggacctgccagagcctgcacatcaatgaaatgtgtcaggagcgatgcgtggatggctgcagctgccctgagggacagctcctggatgaaggcctctgcgtggagagcaccgagtgtccctgcgtgcattccggaaagcgctaccctcccggcacctccctctctcgagactgcaacacctgcatttgccgaaacagccagtggatctgcagcaatgaagaatgtccaggggagtgccttgtcacaggtcaatcacacttcaagagctttgacaacagatacttcaccttcagtgggatctgccagtacctgctggcccgggattgccaggaccactccttctccattgtcattgagactgtccagtgtgctgatgaccgcgacgctgtgtgcacccgctccgtcaccgtccggctgcctggcctgcacaacagccttgtgaaactgaagcatggggcaggagttgccatggatggccaggacgtccagctccccctcctgaaaggtgacctccgcatccagcatacagtgacggcctccgtgcgcctcagctacggggaggacctgcagatggactgggatggccgcgggaggctgctggtgaagctgtcccccgtctatgccgggaagacctgcggcctgtgtgggaattacaatggcaaccagggcgacgacttccttaccccctctgggctggcggagccccgggtggaggacttcgggaacgcctggaagctgcacggggactgccaggacctgcagaagcagcacagcgatccctgcgccctcaacccgcgcatgaccaggttctccgaggaggcgtgcgcggtcctgacgtcccccacattcgaggcctgccatcgtgccgtcagcccgctgccctacctgcggaactgccgctacgacgtgtgctcctgctcggacggccgcgagtgcctgtgcggcgccctggccagctatgccgcggcctgcgcggggagaggcgtgcgcgtcgcgtggcgcgagccaggccgctgtgagctgaactgcccgaaaggccaggtgtacctgcagtgcgggaccccctgcaacctgacctgccgctctctctcttacccggatgaggaatgcaatgaggcctgcctggagggctgcttctgccccccagggctctacatggatgagaggggggactgcgtgcccaaggcccagtgcccctgttactatgacggtgagatcttccagccagaagacatcttctcagaccatcacaccatgtgctactgtgaggatggcttcatgcactgtaccatgagtggagtccccggaagcttgctgcctgacgctgtcctcagcagtcccctgtctcatcgcagcaaaaggagcctatcctgtcggccccccatggtcaagctggtgtgtcccgctgacaacctgcgggctgaagggctcgagtgtaccaaaacgtgccagaactatgacctggagtgcatgagcatgggctgtgtctctggctgcctctgccccccgggcatggtccggcatgagaacagatgtgtggccctggaaaggtgtccctgcttccatcagggcaaggagtatgcccctggagaaacagtgaagattggctgcaacacttgtgtctgtcaggaccggaagtggaactgcacagaccatgtgtgtgatgccacgtgctccacgatcggcatggcccactacctcaccttcgacgggctcaaatacctgttccccggggagtgccagtacgttctggtgcaggattactgcggcagtaaccctgggacctttcggatcctagtggggaataagggatgcagccacccctcagtgaaatgcaagaaacgggtcaccatcctggtggagggaggagagattgagctgtttgacggggaggtgaatgtgaagaggcccatgaaggatgagactcactttgaggtggtggagtctggccggtacatcattctgctgctgggcaaagccctctccgtggtctgggaccgccacctgagcatctccgtggtcctgaagcagacataccaggagaaagtgtgtggcctgtgtgggaattttgatggcatccagaacaatgacctcaccagcagcaacctccaagtggaggaagaccctgtggactttgggaactcctggaaagtgagctcgcagtgtgctgacaccagaaaagtgcctctggactcatcccctgccacctgccataacaacatcatgaagcagacgatggtggattcctcctgtagaatccttaccagtgacgtcttccaggactgcaacaagctggtggaccccgagccatatctggatgtctgcatttacgacacctgctcctgtgagtccattggggactgcgcctgcttctgcgacaccattgctgcctatgcccacgtgtgtgcccagcatggcaaggtggtgacctggaggacggccacattgtgcccccagagctgcgaggagaggaatctccgggagaacgggtatgagtgtgagtggcgctataacagctgtgcacctgcctgtcaagtcacgtgtcagcaccctgagccactggcctgccctgtgcagtgtgtggagggctgccatgcccactgccctccagggaaaatcctggatgagcttttgcagacctgcgttgaccctgaagactgtccagtgtgtgaggtggctggccggcgttttgcctcaggaaagaaagtcaccttgaatcccagtgaccctgagcactgccagatttgccactgtgatgttgtcaacctcacctgtgaagcctgccaggagccgggaggcctggtggtgcctcccacagatgccccggtgagccccaccactctgtatgtggaggacatctcggaaccgccgttgcacgatttctactgcagcaggctactggacctggtcttcctgctggatggctcctccaggctgtccgaggctgagtttgaagtgctgaaggcctttgtggtggacatgatggagcggctgcgcatctcccagaagtgggtccgcgtggccgtggtggagtaccacgacggctcccacgcctacatcgggctcaaggaccggaagcgaccgtcagagctgcggcgcattgccagccaggtgaagtatgcgggcagccaggtggcctccaccagcgaggtcttgaaatacacactgttccaaatcttcagcaagatcgaccgccctgaagcctcccgcatcaccctgctcctgatggccagccaggagccccaacggatgtcccggaactttgtccgctacgtccagggcctgaagaagaagaaggtcattgtgatcccggtgggcattgggccccatgccaacctcaagcagatccgcctcatcgagaagcaggcccctgagaacaaggccttcgtgctgagcagtgtggatgagctggagcagcaaagggacgagatcgttagctacctctgtgaccttgcccctgaagcccctcctcctactctgccccccgacatggcacaagtcactgtgggcccggggctcttgggggtttcgaccctggggcccaagaggaactccatggttctggatgtggcgttcgtcctggaaggatcggacaaaattggtgaagccgacttcaacaggagcaaggagttcatggaggaggtgattcagcggatggatgtgggccaggacagcatccacgtcacggtgctgcagtactcctacatggtgactgtggagtaccccttcagcgaggcacagtccaaaggggacatcctgcagcgggtgcgagagatccgctaccagggcggcaacaggaccaacactgggctggccctgcggtacctctctgaccacagcttcttggtcagccagggtgaccgggagcaggcgcccaacctggtctacatggtcaccggaaatcctgcctctgatgagatcaagaggctgcctggagacatccaggtggtgcccattggagtgggccctaatgccaacgtgcaggagctggagaggattggctggcccaatgcccctatcctcatccaggactttgagacgctcccccgagaggctcctgacctggtgctgcagaggtgctgctccggagaggggctgcagatccccaccctctcccctgcacctgactgcagccagcccctggacgtgatccttctcctggatggctcctccagtttcccagcttcttattttgatgaaatgaagagtttcgccaaggctttcatttcaaaagccaatatagggcctcgtctcactcaggtgtcagtgctgcagtatggaagcatcaccaccattgacgtgccatggaacgtggtcccggagaaagcccatttgctgagccttgtggacgtcatgcagcgggagggaggccccagccaaatcggggatgccttgggctttgctgtgcgatacttgacttcagaaatgcatggtgccaggccgggagcctcaaaggcggtggtcatcctggtcacggacgtctctgtggattcagtggatgcagcagctgatgccgccaggtccaacagagtgacagtgttccctattggaattggagatcgctacgatgcagcccagctacggatcttggcaggcccagcaggcgactccaacgtggtgaagctccagcgaatcgaagacctccctaccatggtcaccttgggcaattccttcctccacaaactgtgctctggatttgttaggatttgcatggatgaggatgggaatgagaagaggcccggggacgtctggaccttgccagaccagtgccacaccgtgacttgccagccagatggccagaccttgctgaagagtcatcgggtcaactgtgaccgggggctgaggccttcgtgccctaacagccagtcccctgttaaagtggaagagacctgtggctgccgctggacctgcccctgcgtgtgcacaggcagctccactcggcacatcgtgacctttgatgggcagaatttcaagctgactggcagctgttcttatgtcctatttcaaaacaaggagcaggacctggaggtgattctccataatggtgcctgcagccctggagcaaggcagggctgcatgaaatccatcgaggtgaagcacagtgccctctccgtcgagctgcacagtgacatggaggtgacggtgaatgggagactggtctctgttccttacgtgggtgggaacatggaagtcaacgtttatggtgccatcatgcatgaggtcagattcaatcaccttggtcacatcttcacattcactccacaaaacaatgagttccaactgcagctcagccccaagacttttgcttcaaagacgtatggtctgtgtgggatctgtgatgagaacggagccaatgacttcatgctgagggatggcacagtcaccacagactggaaaacacttgttcaggaatggactgtgcagcggccagggcagacgtgccagcccatcctggaggagcagtgtcttgtccccgacagctcccactgccaggtcctcctcttaccactgtttgctgaatgccacaaggtcctggctccagccacattctatgccatctgccagcaggacagttgccaccaggagcaagtgtgtgaggtgatcgcctcttatgcccacctctgtcggaccaacggggtctgcgttgactggaggacacctgatttctgtgctatgtcatgcccaccatctctggtctacaaccactgtgagcatggctgtccccggcactgtgatggcaacgtgagctcctgtggggaccatccctccgaaggctgtttctgccctccagataaagtcatgttggaaggcagctgtgtccctgaagaggcctgcactcagtgcattggtgaggatggagtccagcaccagttcctggaagcctgggtcccggaccaccagccctgtcagatctgcacatgcctcagcgggcggaaggtcaactgcacaacgcagccctgccccacggccaaagctcccacgtgtggcctgtgtgaagtagcccgcctccgccagaatgcagaccagtgctgccccgagtatgagtgtgtgtgtgacccagtgagctgtgacctgcccccagtgcctcactgtgaacgtggcctccagcccacactgaccaaccctggcgagtgcagacccaacttcacctgcgcctgcaggaaggaggagtgcaaaagagtgtccccaccctcctgccccccgcaccgtttgcccacccttcggaagacccagtgctgtgatgagtatgagtgtgcctgcaactgtgtcaactccacagtgagctgtccccttgggtacttggcctcaactgccaccaatgactgtggctgtaccacaaccacctgccttcccgacaaggtgtgtgtccaccgaagcaccatctaccctgtgggccagttctgggaggagggctgcgatgtgtgcacctgcaccgacatggaggatgccgtgatgggcctccgcgtggcccagtgctcccagaagccctgtgaggacagctgtcggtcgggcttcacttacgttctgcatgaaggcgagtgctgtggaaggtgcctgccatctgcctgtgaggtggtgactggctcaccgcggggggactcccagtcttcctggaagagtgtcggctcccagtgggcctccccggagaacccctgcctcatcaatgagtgtgtccgagtgaaggaggaggtctttatacaacaaaggaacgtctcctgcccccagctggaggtccctgtctgcccctcgggctttcagctgagctgtaagacctcagcgtgctgcccaagctgtcgctgtgagcgcatggaggcctgcatgctcaatggcactgtcattgggcccgggaagactgtgatgatcgatgtgtgcacgacctgccgctgcatggtgcaggtgggggtcatctctggattcaagctggagtgcaggaagaccacctgcaacccctgccccctgggttacaaggaagaaaataacacaggtgaatgttgtgggagatgtttgcctacggcttgcaccattcagctaagaggaggacagatcatgacactgaagcgtgatgagacgctccaggatggctgtgatactcacttctgcaaggtcaatgagagaggagagtacttctgggagaagagggtcacaggctgcccaccctttgatgaacacaagtgtctggctgagggaggtaaaattatgaaaattccaggcacctgctgtgacacatgtgaggagcctgagtgcaacgacatcactgccaggctgcagtatgtcaaggtgggaagctgtaagtctgaagtagaggtggatatccactactgccagggcaaatgtgccagcaaagccatgtactccattgacatcaacgatgtgcaggaccagtgctcctgctgctctccgacacggacggagcccatgcaggtggccctgcactgcaccaatggctctgttgtgtaccatgaggttctcaatgccatggagtgcaaatgctcccccaggaagtgcagcaagtga